European Patent Application EP 4 725 959 A1, published April 15, 2026. Title: RSV疫苗组合物、方法及其用途. Applicant: 四川三叶草生物制药有限公司. The sequence listing filed with the application follows.

SEQUENCE LISTING (84 sequences)

SEQ ID NO: 1 - protein, 806 aa, synthetic construct
  source 1..806: organism (original language) = 合成构建体
QNITEEFYQSTCSAVSKGYLSALRTGWYTSVITIELSNIKENKCNGTDAKVKLIKQELDKYKNAVTELQLLMQSTPATNNRARRELPRFMNYTLNNAKKTNVTLSKKRKRRFLGFLLGVGSAIASGVAVSKVLHLEGEVNKIKSALLSTNKAVVSLSNGVSVLTSKVLDLKNYIDKQLLPIVNKQSCSISNIATVIEFQQKNNRLLEITREFSVNAGVTTPVSTYMLTNSELLSLINDMPITNDQKKLMSNNVQIVRQQSYSIMSIIKEEVLAYVVQLPLYGVIDTPCWKLHTSPLCTTNTKEGSNICLTRTDRGWYCDNAGSVSFFPQAETCKVQSNRVFCDTMNSLTLPSEVNLCNVDIFNPKYDCKIMTSKTDVSSSVITSLGAIVSCYGKTKCTASNKNRGIIKTFSNGCDYVSNKGVDTVSVGNTLYYVNKQEGKSLYVKGEPIINFYDPLVFPSDEFDASISQVNEKINQSLAFIRKSDELLHNVNAGKRSNGLPGPIGPPGPRGRTGDAGPVGPPGPPGPPGPPGPPSAGFDFSFLPQPPQEKAHDGGRYYRANDANVVRDRDLEVDTTLKSLSQQIENIRSPEGSRKNPARTCRDLKMCHSDWKSGEYWIDPNQGCNLDAIKVFCNMETGETCVYPTQPSVAQKNWYISKNPKDKRHVWFGESMTDGFQFEYGGQGSDPADVAIQLTFLRLMSTEASQNITYHCKNSVAYMDQQTGNLKKALLLQGSNEIEIRAEGNSRFTYSVTVDGCTSHTGAWGKTVIEYKTTKTSRLPIIDVAPLDVGAPDQEFGFDVGPVCFL

SEQ ID NO: 2 - protein, 831 aa, synthetic construct
  source 1..831: organism (original language) = 合成构建体
MELLILKANAITTILTAVTFCFASGQNITEEFYQSTCSAVSKGYLSALRTGWYTSVITIELSNIKENKCNGTDAKVKLIKQELDKYKNAVTELQLLMQSTPATNNRARRELPRFMNYTLNNAKKTNVTLSKKRKRRFLGFLLGVGSAIASGVAVSKVLHLEGEVNKIKSALLSTNKAVVSLSNGVSVLTSKVLDLKNYIDKQLLPIVNKQSCSISNIATVIEFQQKNNRLLEITREFSVNAGVTTPVSTYMLTNSELLSLINDMPITNDQKKLMSNNVQIVRQQSYSIMSIIKEEVLAYVVQLPLYGVIDTPCWKLHTSPLCTTNTKEGSNICLTRTDRGWYCDNAGSVSFFPQAETCKVQSNRVFCDTMNSLTLPSEVNLCNVDIFNPKYDCKIMTSKTDVSSSVITSLGAIVSCYGKTKCTASNKNRGIIKTFSNGCDYVSNKGVDTVSVGNTLYYVNKQEGKSLYVKGEPIINFYDPLVFPSDEFDASISQVNEKINQSLAFIRKSDELLHNVNAGKRSNGLPGPIGPPGPRGRTGDAGPVGPPGPPGPPGPPGPPSAGFDFSFLPQPPQEKAHDGGRYYRANDANVVRDRDLEVDTTLKSLSQQIENIRSPEGSRKNPARTCRDLKMCHSDWKSGEYWIDPNQGCNLDAIKVFCNMETGETCVYPTQPSVAQKNWYISKNPKDKRHVWFGESMTDGFQFEYGGQGSDPADVAIQLTFLRLMSTEASQNITYHCKNSVAYMDQQTGNLKKALLLQGSNEIEIRAEGNSRFTYSVTVDGCTSHTGAWGKTVIEYKTTKTSRLPIIDVAPLDVGAPDQEFGFDVGPVCFL

SEQ ID NO: 3 - protein, 806 aa, synthetic construct
  source 1..806: organism (original language) = 合成构建体
QNITEEFYQSTCSAVSKGYLSALRTGWYTSVITIELSNIKENKCNGTDAKVKLIKQELDKYKNAVTELQLLMQSTPATNNRARAELPRFMNYTLNNAKKTNVTLSKKRKRRFLGFLLGVGSAIASGVAVSKVLHLEGEVNKIKSALLSTNKAVVSLSNGVSVLTSKVLDLKNYIDKQLLPIVNKQSCSISNIATVIEFQQKNNRLLEITREFSVNAGVTTPVSTYMLTNSELLSLINDMPITNDQKKLMSNNVQIVRQQSYSIMSIIKEEVLAYVVQLPLYGVIDTPCWKLHTSPLCTTNTKEGSNICLTRTDRGWYCDNAGSVSFFPQAETCKVQSNRVFCDTMNSLTLPSEVNLCNVDIFNPKYDCKIMTSKTDVSSSVITSLGAIVSCYGKTKCTASNKNRGIIKTFSNGCDYVSNKGVDTVSVGNTLYYVNKQEGKSLYVKGEPIINFYDPLVFPSDEFDASISQVNEKINQSLAFIRKSDELLHNVNAGKRSNGLPGPIGPPGPRGRTGDAGPVGPPGPPGPPGPPGPPSAGFDFSFLPQPPQEKAHDGGRYYRANDANVVRDRDLEVDTTLKSLSQQIENIRSPEGSRKNPARTCRDLKMCHSDWKSGEYWIDPNQGCNLDAIKVFCNMETGETCVYPTQPSVAQKNWYISKNPKDKRHVWFGESMTDGFQFEYGGQGSDPADVAIQLTFLRLMSTEASQNITYHCKNSVAYMDQQTGNLKKALLLQGSNEIEIRAEGNSRFTYSVTVDGCTSHTGAWGKTVIEYKTTKTSRLPIIDVAPLDVGAPDQEFGFDVGPVCFL

SEQ ID NO: 4 - protein, 831 aa, synthetic construct
  source 1..831: organism (original language) = 合成构建体
MELLILKANAITTILTAVTFCFASGQNITEEFYQSTCSAVSKGYLSALRTGWYTSVITIELSNIKENKCNGTDAKVKLIKQELDKYKNAVTELQLLMQSTPATNNRARAELPRFMNYTLNNAKKTNVTLSKKRKRRFLGFLLGVGSAIASGVAVSKVLHLEGEVNKIKSALLSTNKAVVSLSNGVSVLTSKVLDLKNYIDKQLLPIVNKQSCSISNIATVIEFQQKNNRLLEITREFSVNAGVTTPVSTYMLTNSELLSLINDMPITNDQKKLMSNNVQIVRQQSYSIMSIIKEEVLAYVVQLPLYGVIDTPCWKLHTSPLCTTNTKEGSNICLTRTDRGWYCDNAGSVSFFPQAETCKVQSNRVFCDTMNSLTLPSEVNLCNVDIFNPKYDCKIMTSKTDVSSSVITSLGAIVSCYGKTKCTASNKNRGIIKTFSNGCDYVSNKGVDTVSVGNTLYYVNKQEGKSLYVKGEPIINFYDPLVFPSDEFDASISQVNEKINQSLAFIRKSDELLHNVNAGKRSNGLPGPIGPPGPRGRTGDAGPVGPPGPPGPPGPPGPPSAGFDFSFLPQPPQEKAHDGGRYYRANDANVVRDRDLEVDTTLKSLSQQIENIRSPEGSRKNPARTCRDLKMCHSDWKSGEYWIDPNQGCNLDAIKVFCNMETGETCVYPTQPSVAQKNWYISKNPKDKRHVWFGESMTDGFQFEYGGQGSDPADVAIQLTFLRLMSTEASQNITYHCKNSVAYMDQQTGNLKKALLLQGSNEIEIRAEGNSRFTYSVTVDGCTSHTGAWGKTVIEYKTTKTSRLPIIDVAPLDVGAPDQEFGFDVGPVCFL

SEQ ID NO: 5 - protein, 806 aa, synthetic construct
  source 1..806: organism (original language) = 合成构建体
QNITEEFYQSTCSAVSKGYLSALRTGWYTSVITIELSNIKENKCNGTDAKVKLIKQELDKYKNAVTELQLLMQSTPATNNRARRELPRFMNYTLNNAKKTNVTLSKKRKRAFLGFLLGVGSAIASGVAVSKVLHLEGEVNKIKSALLSTNKAVVSLSNGVSVLTSKVLDLKNYIDKQLLPIVNKQSCSISNIATVIEFQQKNNRLLEITREFSVNAGVTTPVSTYMLTNSELLSLINDMPITNDQKKLMSNNVQIVRQQSYSIMSIIKEEVLAYVVQLPLYGVIDTPCWKLHTSPLCTTNTKEGSNICLTRTDRGWYCDNAGSVSFFPQAETCKVQSNRVFCDTMNSLTLPSEVNLCNVDIFNPKYDCKIMTSKTDVSSSVITSLGAIVSCYGKTKCTASNKNRGIIKTFSNGCDYVSNKGVDTVSVGNTLYYVNKQEGKSLYVKGEPIINFYDPLVFPSDEFDASISQVNEKINQSLAFIRKSDELLHNVNAGKRSNGLPGPIGPPGPRGRTGDAGPVGPPGPPGPPGPPGPPSAGFDFSFLPQPPQEKAHDGGRYYRANDANVVRDRDLEVDTTLKSLSQQIENIRSPEGSRKNPARTCRDLKMCHSDWKSGEYWIDPNQGCNLDAIKVFCNMETGETCVYPTQPSVAQKNWYISKNPKDKRHVWFGESMTDGFQFEYGGQGSDPADVAIQLTFLRLMSTEASQNITYHCKNSVAYMDQQTGNLKKALLLQGSNEIEIRAEGNSRFTYSVTVDGCTSHTGAWGKTVIEYKTTKTSRLPIIDVAPLDVGAPDQEFGFDVGPVCFL

SEQ ID NO: 6 - protein, 831 aa, synthetic construct
  source 1..831: organism (original language) = 合成构建体
MELLILKANAITTILTAVTFCFASGQNITEEFYQSTCSAVSKGYLSALRTGWYTSVITIELSNIKENKCNGTDAKVKLIKQELDKYKNAVTELQLLMQSTPATNNRARRELPRFMNYTLNNAKKTNVTLSKKRKRAFLGFLLGVGSAIASGVAVSKVLHLEGEVNKIKSALLSTNKAVVSLSNGVSVLTSKVLDLKNYIDKQLLPIVNKQSCSISNIATVIEFQQKNNRLLEITREFSVNAGVTTPVSTYMLTNSELLSLINDMPITNDQKKLMSNNVQIVRQQSYSIMSIIKEEVLAYVVQLPLYGVIDTPCWKLHTSPLCTTNTKEGSNICLTRTDRGWYCDNAGSVSFFPQAETCKVQSNRVFCDTMNSLTLPSEVNLCNVDIFNPKYDCKIMTSKTDVSSSVITSLGAIVSCYGKTKCTASNKNRGIIKTFSNGCDYVSNKGVDTVSVGNTLYYVNKQEGKSLYVKGEPIINFYDPLVFPSDEFDASISQVNEKINQSLAFIRKSDELLHNVNAGKRSNGLPGPIGPPGPRGRTGDAGPVGPPGPPGPPGPPGPPSAGFDFSFLPQPPQEKAHDGGRYYRANDANVVRDRDLEVDTTLKSLSQQIENIRSPEGSRKNPARTCRDLKMCHSDWKSGEYWIDPNQGCNLDAIKVFCNMETGETCVYPTQPSVAQKNWYISKNPKDKRHVWFGESMTDGFQFEYGGQGSDPADVAIQLTFLRLMSTEASQNITYHCKNSVAYMDQQTGNLKKALLLQGSNEIEIRAEGNSRFTYSVTVDGCTSHTGAWGKTVIEYKTTKTSRLPIIDVAPLDVGAPDQEFGFDVGPVCFL

SEQ ID NO: 7 - protein, 806 aa, synthetic construct
  source 1..806: organism (original language) = 合成构建体
QNITEEFYQSTCSAVSKGYLSALRTGWYTSVITIELSNIKENKCNGTDAKVKLIKQELDKYKNAVTELQLLMQSTPATNNRARAELPRFMNYTLNNAKKTNVTLSKKRKRAFLGFLLGVGSAIASGVAVSKVLHLEGEVNKIKSALLSTNKAVVSLSNGVSVLTSKVLDLKNYIDKQLLPIVNKQSCSISNIATVIEFQQKNNRLLEITREFSVNAGVTTPVSTYMLTNSELLSLINDMPITNDQKKLMSNNVQIVRQQSYSIMSIIKEEVLAYVVQLPLYGVIDTPCWKLHTSPLCTTNTKEGSNICLTRTDRGWYCDNAGSVSFFPQAETCKVQSNRVFCDTMNSLTLPSEVNLCNVDIFNPKYDCKIMTSKTDVSSSVITSLGAIVSCYGKTKCTASNKNRGIIKTFSNGCDYVSNKGVDTVSVGNTLYYVNKQEGKSLYVKGEPIINFYDPLVFPSDEFDASISQVNEKINQSLAFIRKSDELLHNVNAGKRSNGLPGPIGPPGPRGRTGDAGPVGPPGPPGPPGPPGPPSAGFDFSFLPQPPQEKAHDGGRYYRANDANVVRDRDLEVDTTLKSLSQQIENIRSPEGSRKNPARTCRDLKMCHSDWKSGEYWIDPNQGCNLDAIKVFCNMETGETCVYPTQPSVAQKNWYISKNPKDKRHVWFGESMTDGFQFEYGGQGSDPADVAIQLTFLRLMSTEASQNITYHCKNSVAYMDQQTGNLKKALLLQGSNEIEIRAEGNSRFTYSVTVDGCTSHTGAWGKTVIEYKTTKTSRLPIIDVAPLDVGAPDQEFGFDVGPVCFL

SEQ ID NO: 8 - protein, 831 aa, synthetic construct
  source 1..831: organism (original language) = 合成构建体
MELLILKANAITTILTAVTFCFASGQNITEEFYQSTCSAVSKGYLSALRTGWYTSVITIELSNIKENKCNGTDAKVKLIKQELDKYKNAVTELQLLMQSTPATNNRARAELPRFMNYTLNNAKKTNVTLSKKRKRAFLGFLLGVGSAIASGVAVSKVLHLEGEVNKIKSALLSTNKAVVSLSNGVSVLTSKVLDLKNYIDKQLLPIVNKQSCSISNIATVIEFQQKNNRLLEITREFSVNAGVTTPVSTYMLTNSELLSLINDMPITNDQKKLMSNNVQIVRQQSYSIMSIIKEEVLAYVVQLPLYGVIDTPCWKLHTSPLCTTNTKEGSNICLTRTDRGWYCDNAGSVSFFPQAETCKVQSNRVFCDTMNSLTLPSEVNLCNVDIFNPKYDCKIMTSKTDVSSSVITSLGAIVSCYGKTKCTASNKNRGIIKTFSNGCDYVSNKGVDTVSVGNTLYYVNKQEGKSLYVKGEPIINFYDPLVFPSDEFDASISQVNEKINQSLAFIRKSDELLHNVNAGKRSNGLPGPIGPPGPRGRTGDAGPVGPPGPPGPPGPPGPPSAGFDFSFLPQPPQEKAHDGGRYYRANDANVVRDRDLEVDTTLKSLSQQIENIRSPEGSRKNPARTCRDLKMCHSDWKSGEYWIDPNQGCNLDAIKVFCNMETGETCVYPTQPSVAQKNWYISKNPKDKRHVWFGESMTDGFQFEYGGQGSDPADVAIQLTFLRLMSTEASQNITYHCKNSVAYMDQQTGNLKKALLLQGSNEIEIRAEGNSRFTYSVTVDGCTSHTGAWGKTVIEYKTTKTSRLPIIDVAPLDVGAPDQEFGFDVGPVCFL

SEQ ID NO: 9 - protein, 806 aa, synthetic construct
  source 1..806: organism (original language) = 合成构建体
QNITEEFYQSTCSAVSKGYLSALRTGWYTSVITIELSNIKENKCNGTDAKVKLIKQELDKYKNAVTELQLLMQSTPATNNRARRELPRFMNYTLNNAKKTNVTLSKKRKRRFLGFLLGVGSAIASGVAVSKVLHLPGEVNKIKSALLSTNKAVVSLSNGVSVLTSKVLDLKNYIDKQLLPIVNKQSCSIPNIATVIEFQQKNNRLLEITREFSVNAGVTTPVSTYMLTNSELLSLINDMPITNDQKKLMSNNVQIVRQQSYSIMSIIKEEVLAYVVQLPLYGVIDTPCWKLHTSPLCTTNTKEGSNICLTRTDRGWYCDNAGSVSFFPQAETCKVQSNRVFCDTMNSLTLPSEVNLCNVDIFNPKYDCKIMTSKTDVSSSVITSLGAIVSCYGKTKCTASNKNRGIIKTFSNGCDYVSNKGVDTVSVGNTLYYVNKQEGKSLYVKGEPIINFYDPLVFPSDEFDASISQVNEKINQSLAFIRKSDELLHNVNAGKRSNGLPGPIGPPGPRGRTGDAGPVGPPGPPGPPGPPGPPSAGFDFSFLPQPPQEKAHDGGRYYRANDANVVRDRDLEVDTTLKSLSQQIENIRSPEGSRKNPARTCRDLKMCHSDWKSGEYWIDPNQGCNLDAIKVFCNMETGETCVYPTQPSVAQKNWYISKNPKDKRHVWFGESMTDGFQFEYGGQGSDPADVAIQLTFLRLMSTEASQNITYHCKNSVAYMDQQTGNLKKALLLQGSNEIEIRAEGNSRFTYSVTVDGCTSHTGAWGKTVIEYKTTKTSRLPIIDVAPLDVGAPDQEFGFDVGPVCFL

SEQ ID NO: 10 - protein, 831 aa, synthetic construct
  source 1..831: organism (original language) = 合成构建体
MELLILKANAITTILTAVTFCFASGQNITEEFYQSTCSAVSKGYLSALRTGWYTSVITIELSNIKENKCNGTDAKVKLIKQELDKYKNAVTELQLLMQSTPATNNRARRELPRFMNYTLNNAKKTNVTLSKKRKRRFLGFLLGVGSAIASGVAVSKVLHLPGEVNKIKSALLSTNKAVVSLSNGVSVLTSKVLDLKNYIDKQLLPIVNKQSCSIPNIATVIEFQQKNNRLLEITREFSVNAGVTTPVSTYMLTNSELLSLINDMPITNDQKKLMSNNVQIVRQQSYSIMSIIKEEVLAYVVQLPLYGVIDTPCWKLHTSPLCTTNTKEGSNICLTRTDRGWYCDNAGSVSFFPQAETCKVQSNRVFCDTMNSLTLPSEVNLCNVDIFNPKYDCKIMTSKTDVSSSVITSLGAIVSCYGKTKCTASNKNRGIIKTFSNGCDYVSNKGVDTVSVGNTLYYVNKQEGKSLYVKGEPIINFYDPLVFPSDEFDASISQVNEKINQSLAFIRKSDELLHNVNAGKRSNGLPGPIGPPGPRGRTGDAGPVGPPGPPGPPGPPGPPSAGFDFSFLPQPPQEKAHDGGRYYRANDANVVRDRDLEVDTTLKSLSQQIENIRSPEGSRKNPARTCRDLKMCHSDWKSGEYWIDPNQGCNLDAIKVFCNMETGETCVYPTQPSVAQKNWYISKNPKDKRHVWFGESMTDGFQFEYGGQGSDPADVAIQLTFLRLMSTEASQNITYHCKNSVAYMDQQTGNLKKALLLQGSNEIEIRAEGNSRFTYSVTVDGCTSHTGAWGKTVIEYKTTKTSRLPIIDVAPLDVGAPDQEFGFDVGPVCFL

SEQ ID NO: 11 - protein, 806 aa, synthetic construct
  source 1..806: organism (original language) = 合成构建体
QNITEEFYQSTCSAVSKGYLSALRTGWYTSVITIELSNIKENKCNGTDAKVKLIKQELDKYKNAVTELQLLMQSTPATNNRARAELPRFMNYTLNNAKKTNVTLSKKRKRAFLGFLLGVGSAIASGVAVSKVLHLPGEVNKIKSALLSTNKAVVSLSNGVSVLTSKVLDLKNYIDKQLLPIVNKQSCSIPNIATVIEFQQKNNRLLEITREFSVNAGVTTPVSTYMLTNSELLSLINDMPITNDQKKLMSNNVQIVRQQSYSIMSIIKEEVLAYVVQLPLYGVIDTPCWKLHTSPLCTTNTKEGSNICLTRTDRGWYCDNAGSVSFFPQAETCKVQSNRVFCDTMNSLTLPSEVNLCNVDIFNPKYDCKIMTSKTDVSSSVITSLGAIVSCYGKTKCTASNKNRGIIKTFSNGCDYVSNKGVDTVSVGNTLYYVNKQEGKSLYVKGEPIINFYDPLVFPSDEFDASISQVNEKINQSLAFIRKSDELLHNVNAGKRSNGLPGPIGPPGPRGRTGDAGPVGPPGPPGPPGPPGPPSAGFDFSFLPQPPQEKAHDGGRYYRANDANVVRDRDLEVDTTLKSLSQQIENIRSPEGSRKNPARTCRDLKMCHSDWKSGEYWIDPNQGCNLDAIKVFCNMETGETCVYPTQPSVAQKNWYISKNPKDKRHVWFGESMTDGFQFEYGGQGSDPADVAIQLTFLRLMSTEASQNITYHCKNSVAYMDQQTGNLKKALLLQGSNEIEIRAEGNSRFTYSVTVDGCTSHTGAWGKTVIEYKTTKTSRLPIIDVAPLDVGAPDQEFGFDVGPVCFL

SEQ ID NO: 12 - protein, 831 aa, synthetic construct
  source 1..831: organism (original language) = 合成构建体
MELLILKANAITTILTAVTFCFASGQNITEEFYQSTCSAVSKGYLSALRTGWYTSVITIELSNIKENKCNGTDAKVKLIKQELDKYKNAVTELQLLMQSTPATNNRARAELPRFMNYTLNNAKKTNVTLSKKRKRAFLGFLLGVGSAIASGVAVSKVLHLPGEVNKIKSALLSTNKAVVSLSNGVSVLTSKVLDLKNYIDKQLLPIVNKQSCSIPNIATVIEFQQKNNRLLEITREFSVNAGVTTPVSTYMLTNSELLSLINDMPITNDQKKLMSNNVQIVRQQSYSIMSIIKEEVLAYVVQLPLYGVIDTPCWKLHTSPLCTTNTKEGSNICLTRTDRGWYCDNAGSVSFFPQAETCKVQSNRVFCDTMNSLTLPSEVNLCNVDIFNPKYDCKIMTSKTDVSSSVITSLGAIVSCYGKTKCTASNKNRGIIKTFSNGCDYVSNKGVDTVSVGNTLYYVNKQEGKSLYVKGEPIINFYDPLVFPSDEFDASISQVNEKINQSLAFIRKSDELLHNVNAGKRSNGLPGPIGPPGPRGRTGDAGPVGPPGPPGPPGPPGPPSAGFDFSFLPQPPQEKAHDGGRYYRANDANVVRDRDLEVDTTLKSLSQQIENIRSPEGSRKNPARTCRDLKMCHSDWKSGEYWIDPNQGCNLDAIKVFCNMETGETCVYPTQPSVAQKNWYISKNPKDKRHVWFGESMTDGFQFEYGGQGSDPADVAIQLTFLRLMSTEASQNITYHCKNSVAYMDQQTGNLKKALLLQGSNEIEIRAEGNSRFTYSVTVDGCTSHTGAWGKTVIEYKTTKTSRLPIIDVAPLDVGAPDQEFGFDVGPVCFL

SEQ ID NO: 13 - protein, 741 aa, synthetic construct
  source 1..741: organism (original language) = 合成构建体
QNITEEFYQSTCSAVSKGYLSALRTGWYTSVITIELSNIKENKCNGTDAKVKLIKQELDKYKNAVTELQLLMQSTPATNNRARAELPRFMNYTLNNAKKTNVTLSKKRKRAFLGFLLGVGSAIASGVAVSKVLHLPGEVNKIKSALLSTNKAVVSLSNGVSVLTSKVLDLKNYIDKQLLPIVNKQSCSIPNIATVIEFQQKNNRLLEITREFSVNAGVTTPVSTYMLTNSELLSLINDMPITNDQKKLMSNNVQIVRQQSYSIMSIIKEEVLAYVVQLPLYGVIDTPCWKLHTSPLCTTNTKEGSNICLTRTDRGWYCDNAGSVSFFPQAETCKVQSNRVFCDTMNSLTLPSEVNLCNVDIFNPKYDCKIMTSKTDVSSSVITSLGAIVSCYGKTKCTASNKNRGIIKTFSNGCDYVSNKGVDTVSVGNTLYYVNKQEGKSLYVKGEPIINFYDPLVFPSDEFDASISQVNEKINQSLAFIRKSDELLHNVNAGKRSANVVRDRDLEVDTTLKSLSQQIENIRSPEGSRKNPARTCRDLKMCHSDWKSGEYWIDPNQGCNLDAIKVFCNMETGETCVYPTQPSVAQKNWYISKNPKDKRHVWFGESMTDGFQFEYGGQGSDPADVAIQLTFLRLMSTEASQNITYHCKNSVAYMDQQTGNLKKALLLQGSNEIEIRAEGNSRFTYSVTVDGCTSHTGAWGKTVIEYKTTKTSRLPIIDVAPLDVGAPDQEFGFDVGPVCFL

SEQ ID NO: 14 - protein, 766 aa, synthetic construct
  source 1..766: organism (original language) = 合成构建体
MELLILKANAITTILTAVTFCFASGQNITEEFYQSTCSAVSKGYLSALRTGWYTSVITIELSNIKENKCNGTDAKVKLIKQELDKYKNAVTELQLLMQSTPATNNRARAELPRFMNYTLNNAKKTNVTLSKKRKRAFLGFLLGVGSAIASGVAVSKVLHLPGEVNKIKSALLSTNKAVVSLSNGVSVLTSKVLDLKNYIDKQLLPIVNKQSCSIPNIATVIEFQQKNNRLLEITREFSVNAGVTTPVSTYMLTNSELLSLINDMPITNDQKKLMSNNVQIVRQQSYSIMSIIKEEVLAYVVQLPLYGVIDTPCWKLHTSPLCTTNTKEGSNICLTRTDRGWYCDNAGSVSFFPQAETCKVQSNRVFCDTMNSLTLPSEVNLCNVDIFNPKYDCKIMTSKTDVSSSVITSLGAIVSCYGKTKCTASNKNRGIIKTFSNGCDYVSNKGVDTVSVGNTLYYVNKQEGKSLYVKGEPIINFYDPLVFPSDEFDASISQVNEKINQSLAFIRKSDELLHNVNAGKRSANVVRDRDLEVDTTLKSLSQQIENIRSPEGSRKNPARTCRDLKMCHSDWKSGEYWIDPNQGCNLDAIKVFCNMETGETCVYPTQPSVAQKNWYISKNPKDKRHVWFGESMTDGFQFEYGGQGSDPADVAIQLTFLRLMSTEASQNITYHCKNSVAYMDQQTGNLKKALLLQGSNEIEIRAEGNSRFTYSVTVDGCTSHTGAWGKTVIEYKTTKTSRLPIIDVAPLDVGAPDQEFGFDVGPVCFL

SEQ ID NO: 15 - protein, 806 aa, synthetic construct
  source 1..806: organism (original language) = 合成构建体
QNITEEFYQSTCSAVSKGYLSALRTGWYTSVITIELSNIKENKCNGTDAKVKLIKQELDKYKNAVTELQLLMQSTPPTNNRARRELPRFMNYTLNNAKKTNVTLSKKRKRRFLGFLLGVGSAIASGVAVSKVLHLEGEVNKIKSALLSTNKAVVSLSNGVSVLTSKVLDLKNYIDKQLLPIVNKQSCSISNIETVIEFQQKNNRLLEITREFSVNAGVTTPVSTYMLTNSELLSLINDMPITNDQKKLMSNNVQIVRQQSYSIMSIIKEEVLAYVVQLPLYGVIDTPCWKLHTSPLCTTNTKEGSNICLTRTDRGWYCDNAGSVSFFPQAETCKVQSNRVFCDTMNSLTLPSEINLCNVDIFNPKYDCKIMTSKTDVSSSVITSLGAIVSCYGKTKCTASNKNRGIIKTFSNGCDYVSNKGMDTVSVGNTLYYVNKQEGKSLYVKGEPIINFYDPLVFPSDEFDASISQVNEKINQSLAFIRKSDELLHNVNAGKRSNGLPGPIGPPGPRGRTGDAGPVGPPGPPGPPGPPGPPSAGFDFSFLPQPPQEKAHDGGRYYRANDANVVRDRDLEVDTTLKSLSQQIENIRSPEGSRKNPARTCRDLKMCHSDWKSGEYWIDPNQGCNLDAIKVFCNMETGETCVYPTQPSVAQKNWYISKNPKDKRHVWFGESMTDGFQFEYGGQGSDPADVAIQLTFLRLMSTEASQNITYHCKNSVAYMDQQTGNLKKALLLQGSNEIEIRAEGNSRFTYSVTVDGCTSHTGAWGKTVIEYKTTKTSRLPIIDVAPLDVGAPDQEFGFDVGPVCFL

SEQ ID NO: 16 - protein, 831 aa, synthetic construct
  source 1..831: organism (original language) = 合成构建体
MELLILKANAITTILTAVTFCFASGQNITEEFYQSTCSAVSKGYLSALRTGWYTSVITIELSNIKENKCNGTDAKVKLIKQELDKYKNAVTELQLLMQSTPPTNNRARRELPRFMNYTLNNAKKTNVTLSKKRKRRFLGFLLGVGSAIASGVAVSKVLHLEGEVNKIKSALLSTNKAVVSLSNGVSVLTSKVLDLKNYIDKQLLPIVNKQSCSISNIETVIEFQQKNNRLLEITREFSVNAGVTTPVSTYMLTNSELLSLINDMPITNDQKKLMSNNVQIVRQQSYSIMSIIKEEVLAYVVQLPLYGVIDTPCWKLHTSPLCTTNTKEGSNICLTRTDRGWYCDNAGSVSFFPQAETCKVQSNRVFCDTMNSLTLPSEINLCNVDIFNPKYDCKIMTSKTDVSSSVITSLGAIVSCYGKTKCTASNKNRGIIKTFSNGCDYVSNKGMDTVSVGNTLYYVNKQEGKSLYVKGEPIINFYDPLVFPSDEFDASISQVNEKINQSLAFIRKSDELLHNVNAGKRSNGLPGPIGPPGPRGRTGDAGPVGPPGPPGPPGPPGPPSAGFDFSFLPQPPQEKAHDGGRYYRANDANVVRDRDLEVDTTLKSLSQQIENIRSPEGSRKNPARTCRDLKMCHSDWKSGEYWIDPNQGCNLDAIKVFCNMETGETCVYPTQPSVAQKNWYISKNPKDKRHVWFGESMTDGFQFEYGGQGSDPADVAIQLTFLRLMSTEASQNITYHCKNSVAYMDQQTGNLKKALLLQGSNEIEIRAEGNSRFTYSVTVDGCTSHTGAWGKTVIEYKTTKTSRLPIIDVAPLDVGAPDQEFGFDVGPVCFL

SEQ ID NO: 17 - protein, 495 aa, synthetic construct
  source 1..495: organism (original language) = 合成构建体
QNITEEFYQSTCSAVSKGYLSALRTGWYTSVITIELSNIKENKCNGTDAKVKLIKQELDKYKNAVTELQLLMQSTPATNNRARRELPRFMNYTLNNAKKTNVTLSKKRKRRFLGFLLGVGSAIASGVAVSKVLHLEGEVNKIKSALLSTNKAVVSLSNGVSVLTSKVLDLKNYIDKQLLPIVNKQSCSISNIATVIEFQQKNNRLLEITREFSVNAGVTTPVSTYMLTNSELLSLINDMPITNDQKKLMSNNVQIVRQQSYSIMSIIKEEVLAYVVQLPLYGVIDTPCWKLHTSPLCTTNTKEGSNICLTRTDRGWYCDNAGSVSFFPQAETCKVQSNRVFCDTMNSLTLPSEVNLCNVDIFNPKYDCKIMTSKTDVSSSVITSLGAIVSCYGKTKCTASNKNRGIIKTFSNGCDYVSNKGVDTVSVGNTLYYVNKQEGKSLYVKGEPIINFYDPLVFPSDEFDASISQVNEKINQSLAFIRKSDELLHNVNAGK

SEQ ID NO: 18 - protein, 520 aa, synthetic construct
  source 1..520: organism (original language) = 合成构建体
MELLILKANAITTILTAVTFCFASGQNITEEFYQSTCSAVSKGYLSALRTGWYTSVITIELSNIKENKCNGTDAKVKLIKQELDKYKNAVTELQLLMQSTPATNNRARRELPRFMNYTLNNAKKTNVTLSKKRKRRFLGFLLGVGSAIASGVAVSKVLHLEGEVNKIKSALLSTNKAVVSLSNGVSVLTSKVLDLKNYIDKQLLPIVNKQSCSISNIATVIEFQQKNNRLLEITREFSVNAGVTTPVSTYMLTNSELLSLINDMPITNDQKKLMSNNVQIVRQQSYSIMSIIKEEVLAYVVQLPLYGVIDTPCWKLHTSPLCTTNTKEGSNICLTRTDRGWYCDNAGSVSFFPQAETCKVQSNRVFCDTMNSLTLPSEVNLCNVDIFNPKYDCKIMTSKTDVSSSVITSLGAIVSCYGKTKCTASNKNRGIIKTFSNGCDYVSNKGVDTVSVGNTLYYVNKQEGKSLYVKGEPIINFYDPLVFPSDEFDASISQVNEKINQSLAFIRKSDELLHNVNAGK

SEQ ID NO: 19 - protein, 495 aa, synthetic construct
  source 1..495: organism (original language) = 合成构建体
QNITEEFYQSTCSAVSKGYLSALRTGWYTSVITIELSNIKENKCNGTDAKVKLIKQELDKYKNAVTELQLLMQSTPATNNRARAELPRFMNYTLNNAKKTNVTLSKKRKRRFLGFLLGVGSAIASGVAVSKVLHLEGEVNKIKSALLSTNKAVVSLSNGVSVLTSKVLDLKNYIDKQLLPIVNKQSCSISNIATVIEFQQKNNRLLEITREFSVNAGVTTPVSTYMLTNSELLSLINDMPITNDQKKLMSNNVQIVRQQSYSIMSIIKEEVLAYVVQLPLYGVIDTPCWKLHTSPLCTTNTKEGSNICLTRTDRGWYCDNAGSVSFFPQAETCKVQSNRVFCDTMNSLTLPSEVNLCNVDIFNPKYDCKIMTSKTDVSSSVITSLGAIVSCYGKTKCTASNKNRGIIKTFSNGCDYVSNKGVDTVSVGNTLYYVNKQEGKSLYVKGEPIINFYDPLVFPSDEFDASISQVNEKINQSLAFIRKSDELLHNVNAGK

SEQ ID NO: 20 - protein, 520 aa, synthetic construct
  source 1..520: organism (original language) = 合成构建体
MELLILKANAITTILTAVTFCFASGQNITEEFYQSTCSAVSKGYLSALRTGWYTSVITIELSNIKENKCNGTDAKVKLIKQELDKYKNAVTELQLLMQSTPATNNRARAELPRFMNYTLNNAKKTNVTLSKKRKRRFLGFLLGVGSAIASGVAVSKVLHLEGEVNKIKSALLSTNKAVVSLSNGVSVLTSKVLDLKNYIDKQLLPIVNKQSCSISNIATVIEFQQKNNRLLEITREFSVNAGVTTPVSTYMLTNSELLSLINDMPITNDQKKLMSNNVQIVRQQSYSIMSIIKEEVLAYVVQLPLYGVIDTPCWKLHTSPLCTTNTKEGSNICLTRTDRGWYCDNAGSVSFFPQAETCKVQSNRVFCDTMNSLTLPSEVNLCNVDIFNPKYDCKIMTSKTDVSSSVITSLGAIVSCYGKTKCTASNKNRGIIKTFSNGCDYVSNKGVDTVSVGNTLYYVNKQEGKSLYVKGEPIINFYDPLVFPSDEFDASISQVNEKINQSLAFIRKSDELLHNVNAGK

SEQ ID NO: 21 - protein, 806 aa, synthetic construct; identical to SEQ ID NO: 5
  source 1..806: organism (original language) = 合成构建体

SEQ ID NO: 22 - protein, 520 aa, synthetic construct
  source 1..520: organism (original language) = 合成构建体
MELLILKANAITTILTAVTFCFASGQNITEEFYQSTCSAVSKGYLSALRTGWYTSVITIELSNIKENKCNGTDAKVKLIKQELDKYKNAVTELQLLMQSTPATNNRARRELPRFMNYTLNNAKKTNVTLSKKRKRAFLGFLLGVGSAIASGVAVSKVLHLEGEVNKIKSALLSTNKAVVSLSNGVSVLTSKVLDLKNYIDKQLLPIVNKQSCSISNIATVIEFQQKNNRLLEITREFSVNAGVTTPVSTYMLTNSELLSLINDMPITNDQKKLMSNNVQIVRQQSYSIMSIIKEEVLAYVVQLPLYGVIDTPCWKLHTSPLCTTNTKEGSNICLTRTDRGWYCDNAGSVSFFPQAETCKVQSNRVFCDTMNSLTLPSEVNLCNVDIFNPKYDCKIMTSKTDVSSSVITSLGAIVSCYGKTKCTASNKNRGIIKTFSNGCDYVSNKGVDTVSVGNTLYYVNKQEGKSLYVKGEPIINFYDPLVFPSDEFDASISQVNEKINQSLAFIRKSDELLHNVNAGK

SEQ ID NO: 23 - protein, 495 aa, synthetic construct
  source 1..495: organism (original language) = 合成构建体
QNITEEFYQSTCSAVSKGYLSALRTGWYTSVITIELSNIKENKCNGTDAKVKLIKQELDKYKNAVTELQLLMQSTPATNNRARAELPRFMNYTLNNAKKTNVTLSKKRKRAFLGFLLGVGSAIASGVAVSKVLHLEGEVNKIKSALLSTNKAVVSLSNGVSVLTSKVLDLKNYIDKQLLPIVNKQSCSISNIATVIEFQQKNNRLLEITREFSVNAGVTTPVSTYMLTNSELLSLINDMPITNDQKKLMSNNVQIVRQQSYSIMSIIKEEVLAYVVQLPLYGVIDTPCWKLHTSPLCTTNTKEGSNICLTRTDRGWYCDNAGSVSFFPQAETCKVQSNRVFCDTMNSLTLPSEVNLCNVDIFNPKYDCKIMTSKTDVSSSVITSLGAIVSCYGKTKCTASNKNRGIIKTFSNGCDYVSNKGVDTVSVGNTLYYVNKQEGKSLYVKGEPIINFYDPLVFPSDEFDASISQVNEKINQSLAFIRKSDELLHNVNAGK

SEQ ID NO: 24 - protein, 520 aa, synthetic construct
  source 1..520: organism (original language) = 合成构建体
MELLILKANAITTILTAVTFCFASGQNITEEFYQSTCSAVSKGYLSALRTGWYTSVITIELSNIKENKCNGTDAKVKLIKQELDKYKNAVTELQLLMQSTPATNNRARAELPRFMNYTLNNAKKTNVTLSKKRKRAFLGFLLGVGSAIASGVAVSKVLHLEGEVNKIKSALLSTNKAVVSLSNGVSVLTSKVLDLKNYIDKQLLPIVNKQSCSISNIATVIEFQQKNNRLLEITREFSVNAGVTTPVSTYMLTNSELLSLINDMPITNDQKKLMSNNVQIVRQQSYSIMSIIKEEVLAYVVQLPLYGVIDTPCWKLHTSPLCTTNTKEGSNICLTRTDRGWYCDNAGSVSFFPQAETCKVQSNRVFCDTMNSLTLPSEVNLCNVDIFNPKYDCKIMTSKTDVSSSVITSLGAIVSCYGKTKCTASNKNRGIIKTFSNGCDYVSNKGVDTVSVGNTLYYVNKQEGKSLYVKGEPIINFYDPLVFPSDEFDASISQVNEKINQSLAFIRKSDELLHNVNAGK

SEQ ID NO: 25 - protein, 495 aa, synthetic construct
  source 1..495: organism (original language) = 合成构建体
QNITEEFYQSTCSAVSKGYLSALRTGWYTSVITIELSNIKENKCNGTDAKVKLIKQELDKYKNAVTELQLLMQSTPATNNRARRELPRFMNYTLNNAKKTNVTLSKKRKRRFLGFLLGVGSAIASGVAVSKVLHLPGEVNKIKSALLSTNKAVVSLSNGVSVLTSKVLDLKNYIDKQLLPIVNKQSCSIPNIATVIEFQQKNNRLLEITREFSVNAGVTTPVSTYMLTNSELLSLINDMPITNDQKKLMSNNVQIVRQQSYSIMSIIKEEVLAYVVQLPLYGVIDTPCWKLHTSPLCTTNTKEGSNICLTRTDRGWYCDNAGSVSFFPQAETCKVQSNRVFCDTMNSLTLPSEVNLCNVDIFNPKYDCKIMTSKTDVSSSVITSLGAIVSCYGKTKCTASNKNRGIIKTFSNGCDYVSNKGVDTVSVGNTLYYVNKQEGKSLYVKGEPIINFYDPLVFPSDEFDASISQVNEKINQSLAFIRKSDELLHNVNAGK

SEQ ID NO: 26 - protein, 520 aa, synthetic construct
  source 1..520: organism (original language) = 合成构建体
MELLILKANAITTILTAVTFCFASGQNITEEFYQSTCSAVSKGYLSALRTGWYTSVITIELSNIKENKCNGTDAKVKLIKQELDKYKNAVTELQLLMQSTPATNNRARRELPRFMNYTLNNAKKTNVTLSKKRKRRFLGFLLGVGSAIASGVAVSKVLHLPGEVNKIKSALLSTNKAVVSLSNGVSVLTSKVLDLKNYIDKQLLPIVNKQSCSIPNIATVIEFQQKNNRLLEITREFSVNAGVTTPVSTYMLTNSELLSLINDMPITNDQKKLMSNNVQIVRQQSYSIMSIIKEEVLAYVVQLPLYGVIDTPCWKLHTSPLCTTNTKEGSNICLTRTDRGWYCDNAGSVSFFPQAETCKVQSNRVFCDTMNSLTLPSEVNLCNVDIFNPKYDCKIMTSKTDVSSSVITSLGAIVSCYGKTKCTASNKNRGIIKTFSNGCDYVSNKGVDTVSVGNTLYYVNKQEGKSLYVKGEPIINFYDPLVFPSDEFDASISQVNEKINQSLAFIRKSDELLHNVNAGK

SEQ ID NO: 27 - protein, 495 aa, synthetic construct
  source 1..495: organism (original language) = 合成构建体
QNITEEFYQSTCSAVSKGYLSALRTGWYTSVITIELSNIKENKCNGTDAKVKLIKQELDKYKNAVTELQLLMQSTPATNNRARAELPRFMNYTLNNAKKTNVTLSKKRKRAFLGFLLGVGSAIASGVAVSKVLHLPGEVNKIKSALLSTNKAVVSLSNGVSVLTSKVLDLKNYIDKQLLPIVNKQSCSIPNIATVIEFQQKNNRLLEITREFSVNAGVTTPVSTYMLTNSELLSLINDMPITNDQKKLMSNNVQIVRQQSYSIMSIIKEEVLAYVVQLPLYGVIDTPCWKLHTSPLCTTNTKEGSNICLTRTDRGWYCDNAGSVSFFPQAETCKVQSNRVFCDTMNSLTLPSEVNLCNVDIFNPKYDCKIMTSKTDVSSSVITSLGAIVSCYGKTKCTASNKNRGIIKTFSNGCDYVSNKGVDTVSVGNTLYYVNKQEGKSLYVKGEPIINFYDPLVFPSDEFDASISQVNEKINQSLAFIRKSDELLHNVNAGK

SEQ ID NO: 28 - protein, 520 aa, synthetic construct
  source 1..520: organism (original language) = 合成构建体
MELLILKANAITTILTAVTFCFASGQNITEEFYQSTCSAVSKGYLSALRTGWYTSVITIELSNIKENKCNGTDAKVKLIKQELDKYKNAVTELQLLMQSTPATNNRARAELPRFMNYTLNNAKKTNVTLSKKRKRAFLGFLLGVGSAIASGVAVSKVLHLPGEVNKIKSALLSTNKAVVSLSNGVSVLTSKVLDLKNYIDKQLLPIVNKQSCSIPNIATVIEFQQKNNRLLEITREFSVNAGVTTPVSTYMLTNSELLSLINDMPITNDQKKLMSNNVQIVRQQSYSIMSIIKEEVLAYVVQLPLYGVIDTPCWKLHTSPLCTTNTKEGSNICLTRTDRGWYCDNAGSVSFFPQAETCKVQSNRVFCDTMNSLTLPSEVNLCNVDIFNPKYDCKIMTSKTDVSSSVITSLGAIVSCYGKTKCTASNKNRGIIKTFSNGCDYVSNKGVDTVSVGNTLYYVNKQEGKSLYVKGEPIINFYDPLVFPSDEFDASISQVNEKINQSLAFIRKSDELLHNVNAGK

SEQ ID NO: 29 - protein, 495 aa, synthetic construct
  source 1..495: organism (original language) = 合成构建体
QNITEEFYQSTCSAVSKGYLSALRTGWYTSVITIELSNIKENKCNGTDAKVKLIKQELDKYKNAVTELQLLMQSTPPTNNRARRELPRFMNYTLNNAKKTNVTLSKKRKRRFLGFLLGVGSAIASGVAVSKVLHLEGEVNKIKSALLSTNKAVVSLSNGVSVLTSKVLDLKNYIDKQLLPIVNKQSCSISNIETVIEFQQKNNRLLEITREFSVNAGVTTPVSTYMLTNSELLSLINDMPITNDQKKLMSNNVQIVRQQSYSIMSIIKEEVLAYVVQLPLYGVIDTPCWKLHTSPLCTTNTKEGSNICLTRTDRGWYCDNAGSVSFFPQAETCKVQSNRVFCDTMNSLTLPSEINLCNVDIFNPKYDCKIMTSKTDVSSSVITSLGAIVSCYGKTKCTASNKNRGIIKTFSNGCDYVSNKGMDTVSVGNTLYYVNKQEGKSLYVKGEPIINFYDPLVFPSDEFDASISQVNEKINQSLAFIRKSDELLHNVNAGK

SEQ ID NO: 30 - protein, 520 aa, synthetic construct
  source 1..520: organism (original language) = 合成构建体
MELLILKANAITTILTAVTFCFASGQNITEEFYQSTCSAVSKGYLSALRTGWYTSVITIELSNIKENKCNGTDAKVKLIKQELDKYKNAVTELQLLMQSTPPTNNRARRELPRFMNYTLNNAKKTNVTLSKKRKRRFLGFLLGVGSAIASGVAVSKVLHLEGEVNKIKSALLSTNKAVVSLSNGVSVLTSKVLDLKNYIDKQLLPIVNKQSCSISNIETVIEFQQKNNRLLEITREFSVNAGVTTPVSTYMLTNSELLSLINDMPITNDQKKLMSNNVQIVRQQSYSIMSIIKEEVLAYVVQLPLYGVIDTPCWKLHTSPLCTTNTKEGSNICLTRTDRGWYCDNAGSVSFFPQAETCKVQSNRVFCDTMNSLTLPSEINLCNVDIFNPKYDCKIMTSKTDVSSSVITSLGAIVSCYGKTKCTASNKNRGIIKTFSNGCDYVSNKGMDTVSVGNTLYYVNKQEGKSLYVKGEPIINFYDPLVFPSDEFDASISQVNEKINQSLAFIRKSDELLHNVNAGK

SEQ ID NO: 31 - protein, 574 aa, synthetic construct
  source 1..574: organism (original language) = 合成构建体
MELLILKANAITTILTAVTFCFASGQNITEEFYQSTCSAVSKGYLSALRTGWYTSVITIELSNIKENKCNGTDAKVKLIKQELDKYKNAVTELQLLMQSTPPTNNRARRELPRFMNYTLNNAKKTNVTLSKKRKRRFLGFLLGVGSAIASGVAVSKVLHLEGEVNKIKSALLSTNKAVVSLSNGVSVLTSKVLDLKNYIDKQLLPIVNKQSCSISNIETVIEFQQKNNRLLEITREFSVNAGVTTPVSTYMLTNSELLSLINDMPITNDQKKLMSNNVQIVRQQSYSIMSIIKEEVLAYVVQLPLYGVIDTPCWKLHTSPLCTTNTKEGSNICLTRTDRGWYCDNAGSVSFFPQAETCKVQSNRVFCDTMNSLTLPSEINLCNVDIFNPKYDCKIMTSKTDVSSSVITSLGAIVSCYGKTKCTASNKNRGIIKTFSNGCDYVSNKGMDTVSVGNTLYYVNKQEGKSLYVKGEPIINFYDPLVFPSDEFDASISQVNEKINQSLAFIRKSDELLHNVNAGKSTTNIMITTIIIVIIVILLSLIAVGLLLYCKARSTPVTLSKDQLSGINNIAFSN

SEQ ID NO: 32 - protein, 574 aa, synthetic construct
  source 1..574: organism (original language) = 合成构建体
MELLILKANAITTILTAVTFCFASGQNITEEFYQSTCSAVSKGYLSALRTGWYTSVITIELSNIKENKCNGTDAKVKLIKQELDKYKNAVTELQLLMQSTPATNNRARRELPRFMNYTLNNAKKTNVTLSKKRKRRFLGFLLGVGSAIASGVAVSKVLHLEGEVNKIKSALLSTNKAVVSLSNGVSVLTSKVLDLKNYIDKQLLPIVNKQSCSISNIATVIEFQQKNNRLLEITREFSVNAGVTTPVSTYMLTNSELLSLINDMPITNDQKKLMSNNVQIVRQQSYSIMSIIKEEVLAYVVQLPLYGVIDTPCWKLHTSPLCTTNTKEGSNICLTRTDRGWYCDNAGSVSFFPQAETCKVQSNRVFCDTMNSLTLPSEVNLCNVDIFNPKYDCKIMTSKTDVSSSVITSLGAIVSCYGKTKCTASNKNRGIIKTFSNGCDYVSNKGVDTVSVGNTLYYVNKQEGKSLYVKGEPIINFYDPLVFPSDEFDASISQVNEKINQSLAFIRKSDELLHNVNAGKSTTNIMITTIIIVIIVILLSLIAVGLLLYCKARSTPVTLSKDQLSGINNIAFSN

SEQ ID NO: 33 - protein, 25 aa, synthetic construct
  source 1..25: organism (original language) = 合成构建体
MELLILKANAITTILTAVTFCFASG

SEQ ID NO: 34 - protein, 84 aa, synthetic construct
  source 1..84: organism (original language) = 合成构建体
QNITEEFYQSTCSAVSKGYLSALRTGWYTSVITIELSNIKENKCNGTDAKVKLIKQELDKYKNAVTELQLLMQSTPPTNNRARR

SEQ ID NO: 35 - protein, 84 aa, synthetic construct
  source 1..84: organism (original language) = 合成构建体
QNITEEFYQSTCSAVSKGYLSALRTGWYTSVITIELSNIKENKCNGTDAKVKLIKQELDKYKNAVTELQLLMQSTPATNNRARR

SEQ ID NO: 36 - protein, 4 aa, synthetic construct
  source 1..4: organism (original language) = 合成构建体
RARR

SEQ ID NO: 37 - protein, 4 aa, synthetic construct
  source 1..4: organism (original language) = 合成构建体
RARA

SEQ ID NO: 38 - protein, 27 aa, synthetic construct
  source 1..27: organism (original language) = 合成构建体
ELPRFMNYTLNNAKKTNVTLSKKRKRR

SEQ ID NO: 39 - protein, 6 aa, synthetic construct
  source 1..6: organism (original language) = 合成构建体
KKRKRR

SEQ ID NO: 40 - protein, 6 aa, synthetic construct
  source 1..6: organism (original language) = 合成构建体
KKRKRA

SEQ ID NO: 41 - protein, 19 aa, synthetic construct
  source 1..19: organism (original language) = 合成构建体
FLGFLLGVGSAIASGVAVS

SEQ ID NO: 42 - protein, 388 aa, synthetic construct
  source 1..388: organism (original language) = 合成构建体
FLGFLLGVGSAIASGVAVSKVLHLEGEVNKIKSALLSTNKAVVSLSNGVSVLTSKVLDLKNYIDKQLLPIVNKQSCSISNIETVIEFQQKNNRLLEITREFSVNAGVTTPVSTYMLTNSELLSLINDMPITNDQKKLMSNNVQIVRQQSYSIMSIIKEEVLAYVVQLPLYGVIDTPCWKLHTSPLCTTNTKEGSNICLTRTDRGWYCDNAGSVSFFPQAETCKVQSNRVFCDTMNSLTLPSEINLCNVDIFNPKYDCKIMTSKTDVSSSVITSLGAIVSCYGKTKCTASNKNRGIIKTFSNGCDYVSNKGMDTVSVGNTLYYVNKQEGKSLYVKGEPIINFYDPLVFPSDEFDASISQVNEKINQSLAFIRKSDELLHNVNAGKSTTN

SEQ ID NO: 43 - protein, 388 aa, synthetic construct
  source 1..388: organism (original language) = 合成构建体
FLGFLLGVGSAIASGVAVSKVLHLEGEVNKIKSALLSTNKAVVSLSNGVSVLTSKVLDLKNYIDKQLLPIVNKQSCSISNIATVIEFQQKNNRLLEITREFSVNAGVTTPVSTYMLTNSELLSLINDMPITNDQKKLMSNNVQIVRQQSYSIMSIIKEEVLAYVVQLPLYGVIDTPCWKLHTSPLCTTNTKEGSNICLTRTDRGWYCDNAGSVSFFPQAETCKVQSNRVFCDTMNSLTLPSEVNLCNVDIFNPKYDCKIMTSKTDVSSSVITSLGAIVSCYGKTKCTASNKNRGIIKTFSNGCDYVSNKGVDTVSVGNTLYYVNKQEGKSLYVKGEPIINFYDPLVFPSDEFDASISQVNEKINQSLAFIRKSDELLHNVNAGKSTTN

SEQ ID NO: 44 - protein, 26 aa, synthetic construct
  source 1..26: organism (original language) = 合成构建体
IMITTIIIVIIVILLSLIAVGLLLYC

SEQ ID NO: 45 - protein, 24 aa, synthetic construct
  source 1..24: organism (original language) = 合成构建体
KARSTPVTLSKDQLSGINNIAFSN

SEQ ID NO: 46 - protein, 365 aa, synthetic construct
  source 1..365: organism (original language) = 合成构建体
KVLHLEGEVNKIKSALLSTNKAVVSLSNGVSVLTSKVLDLKNYIDKQLLPIVNKQSCSISNIETVIEFQQKNNRLLEITREFSVNAGVTTPVSTYMLTNSELLSLINDMPITNDQKKLMSNNVQIVRQQSYSIMSIIKEEVLAYVVQLPLYGVIDTPCWKLHTSPLCTTNTKEGSNICLTRTDRGWYCDNAGSVSFFPQAETCKVQSNRVFCDTMNSLTLPSEINLCNVDIFNPKYDCKIMTSKTDVSSSVITSLGAIVSCYGKTKCTASNKNRGIIKTFSNGCDYVSNKGMDTVSVGNTLYYVNKQEGKSLYVKGEPIINFYDPLVFPSDEFDASISQVNEKINQSLAFIRKSDELLHNVNAGK

SEQ ID NO: 47 - protein, 365 aa, synthetic construct
  source 1..365: organism (original language) = 合成构建体
KVLHLEGEVNKIKSALLSTNKAVVSLSNGVSVLTSKVLDLKNYIDKQLLPIVNKQSCSISNIATVIEFQQKNNRLLEITREFSVNAGVTTPVSTYMLTNSELLSLINDMPITNDQKKLMSNNVQIVRQQSYSIMSIIKEEVLAYVVQLPLYGVIDTPCWKLHTSPLCTTNTKEGSNICLTRTDRGWYCDNAGSVSFFPQAETCKVQSNRVFCDTMNSLTLPSEVNLCNVDIFNPKYDCKIMTSKTDVSSSVITSLGAIVSCYGKTKCTASNKNRGIIKTFSNGCDYVSNKGVDTVSVGNTLYYVNKQEGKSLYVKGEPIINFYDPLVFPSDEFDASISQVNEKINQSLAFIRKSDELLHNVNAGK

SEQ ID NO: 48 - protein, 244 aa, synthetic construct
  source 1..244: organism (original language) = 合成构建体
ANVVRDRDLEVDTTLKSLSQQIENIRSPEGSRKNPARTCRDLKMCHSDWKSGEYWIDPNQGCNLDAIKVFCNMETGETCVYPTQPSVAQKNWYISKNPKDKRHVWFGESMTDGFQFEYGGQGSDPADVAIQLTFLRLMSTEASQNITYHCKNSVAYMDQQTGNLKKALLLQGSNEIEIRAEGNSRFTYSVTVDGCTSHTGAWGKTVIEYKTTKTSRLPIIDVAPLDVGAPDQEFGFDVGPVCFL

SEQ ID NO: 49 - protein, 246 aa, synthetic construct
  source 1..246: organism (original language) = 合成构建体
RSANVVRDRDLEVDTTLKSLSQQIENIRSPEGSRKNPARTCRDLKMCHSDWKSGEYWIDPNQGCNLDAIKVFCNMETGETCVYPTQPSVAQKNWYISKNPKDKRHVWFGESMTDGFQFEYGGQGSDPADVAIQLTFLRLMSTEASQNITYHCKNSVAYMDQQTGNLKKALLLQGSNEIEIRAEGNSRFTYSVTVDGCTSHTGAWGKTVIEYKTTKTSRLPIIDVAPLDVGAPDQEFGFDVGPVCFL

SEQ ID NO: 50 - protein, 309 aa, synthetic construct
  source 1..309: organism (original language) = 合成构建体
NGLPGPIGPPGPRGRTGDAGPVGPPGPPGPPGPPGPPSAGFDFSFLPQPPQEKAHDGGRYYRANDANVVRDRDLEVDTTLKSLSQQIENIRSPEGSRKNPARTCRDLKMCHSDWKSGEYWIDPNQGCNLDAIKVFCNMETGETCVYPTQPSVAQKNWYISKNPKDKRHVWFGESMTDGFQFEYGGQGSDPADVAIQLTFLRLMSTEASQNITYHCKNSVAYMDQQTGNLKKALLLQGSNEIEIRAEGNSRFTYSVTVDGCTSHTGAWGKTVIEYKTTKTSRLPIIDVAPLDVGAPDQEFGFDVGPVCFL

SEQ ID NO: 51 - protein, 309 aa, synthetic construct
  source 1..309: organism (original language) = 合成构建体
NGLPGPIGPPGPRGRTGDAGPVGPPGPPGPPGPPGPPSAGFDFSFLPQPPQEKAHDGGRYYRNDDANVVRDRDLEVDTTLKSLSQQIENIRSPEGSRKNPARTCRDLKMCHSDWKSGEYWIDPNQGCNLDAIKVFCNMETGETCVYPTQPSVAQKNWYISKNPKDKRHVWFGESMTDGFQFEYGGQGSDPADVAIQLTFLRLMSTEASQNITYHCKNSVAYMDQQTGNLKKALLLQGSNEIEIRAEGNSRFTYSVTVDGCTSHTGAWGKTVIEYKTTKTSRLPIIDVAPLDVGAPDQEFGFDVGPVCFL

SEQ ID NO: 52 - protein, 311 aa, synthetic construct
  source 1..311: organism (original language) = 合成构建体
RSNGLPGPIGPPGPRGRTGDAGPVGPPGPPGPPGPPGPPSAGFDFSFLPQPPQEKAHDGGRYYRANDANVVRDRDLEVDTTLKSLSQQIENIRSPEGSRKNPARTCRDLKMCHSDWKSGEYWIDPNQGCNLDAIKVFCNMETGETCVYPTQPSVAQKNWYISKNPKDKRHVWFGESMTDGFQFEYGGQGSDPADVAIQLTFLRLMSTEASQNITYHCKNSVAYMDQQTGNLKKALLLQGSNEIEIRAEGNSRFTYSVTVDGCTSHTGAWGKTVIEYKTTKTSRLPIIDVAPLDVGAPDQEFGFDVGPVCFL

SEQ ID NO: 53 - protein, 311 aa, synthetic construct
  source 1..311: organism (original language) = 合成构建体
GSNGLPGPIGPPGPRGRTGDAGPVGPPGPPGPPGPPGPPSAGFDFSFLPQPPQEKAHDGGRYYRANDANVVRDRDLEVDTTLKSLSQQIENIRSPEGSRKNPARTCRDLKMCHSDWKSGEYWIDPNQGCNLDAIKVFCNMETGETCVYPTQPSVAQKNWYISKNPKDKRHVWFGESMTDGFQFEYGGQGSDPADVAIQLTFLRLMSTEASQNITYHCKNSVAYMDQQTGNLKKALLLQGSNEIEIRAEGNSRFTYSVTVDGCTSHTGAWGKTVIEYKTTKTSRLPIIDVAPLDVGAPDQEFGFDVGPVCFL

SEQ ID NO: 54 - protein, 244 aa, synthetic construct
  source 1..244: organism (original language) = 合成构建体
ANVVRDRDLEVDTTLKSLSQQIENIRSPEGSRKNPARTCRDLKMCHSDWKSGEYWIDPNQGCNLDAIKVFCNMETGETCVYPTQPSVAQKNWYISKNPKDKRHVWFGESMTDGFQFEYGGQGSDPADVAIQLTFLRLMSTEASQNITYHCKNSVAYMDQQTGNLKKALLLKGSNEIEIRAEGNSRFTYSVTVDGCTSHTGAWGKTVIEYKTTKSSRLPIIDVAPLDVGAPDQEFGFDVGPVCFL

SEQ ID NO: 55 - protein, 246 aa, synthetic construct
  source 1..246: organism (original language) = 合成构建体
RSANVVRDRDLEVDTTLKSLSQQIENIRSPEGSRKNPARTCRDLKMCHSDWKSGEYWIDPNQGCNLDAIKVFCNMETGETCVYPTQPSVAQKNWYISKNPKDKRHVWFGESMTDGFQFEYGGQGSDPADVAIQLTFLRLMSTEASQNITYHCKNSVAYMDQQTGNLKKALLLKGSNEIEIRAEGNSRFTYSVTVDGCTSHTGAWGKTVIEYKTTKSSRLPIIDVAPLDVGAPDQEFGFDVGPVCFL

SEQ ID NO: 56 - protein, 309 aa, synthetic construct
  source 1..309: organism (original language) = 合成构建体
NGLPGPIGPPGPRGRTGDAGPVGPPGPPGPPGPPGPPSAGFDFSFLPQPPQEKAHDGGRYYRANDANVVRDRDLEVDTTLKSLSQQIENIRSPEGSRKNPARTCRDLKMCHSDWKSGEYWIDPNQGCNLDAIKVFCNMETGETCVYPTQPSVAQKNWYISKNPKDKRHVWFGESMTDGFQFEYGGQGSDPADVAIQLTFLRLMSTEASQNITYHCKNSVAYMDQQTGNLKKALLLKGSNEIEIRAEGNSRFTYSVTVDGCTSHTGAWGKTVIEYKTTKSSRLPIIDVAPLDVGAPDQEFGFDVGPVCFL

SEQ ID NO: 57 - protein, 309 aa, synthetic construct
  source 1..309: organism (original language) = 合成构建体
NGLPGPIGPPGPRGRTGDAGPVGPPGPPGPPGPPGPPSAGFDFSFLPQPPQEKAHDGGRYYRNDDANVVRDRDLEVDTTLKSLSQQIENIRSPEGSRKNPARTCRDLKMCHSDWKSGEYWIDPNQGCNLDAIKVFCNMETGETCVYPTQPSVAQKNWYISKNPKDKRHVWFGESMTDGFQFEYGGQGSDPADVAIQLTFLRLMSTEASQNITYHCKNSVAYMDQQTGNLKKALLLKGSNEIEIRAEGNSRFTYSVTVDGCTSHTGAWGKTVIEYKTTKSSRLPIIDVAPLDVGAPDQEFGFDVGPVCFL

SEQ ID NO: 58 - protein, 311 aa, synthetic construct
  source 1..311: organism (original language) = 合成构建体
RSNGLPGPIGPPGPRGRTGDAGPVGPPGPPGPPGPPGPPSAGFDFSFLPQPPQEKAHDGGRYYRANDANVVRDRDLEVDTTLKSLSQQIENIRSPEGSRKNPARTCRDLKMCHSDWKSGEYWIDPNQGCNLDAIKVFCNMETGETCVYPTQPSVAQKNWYISKNPKDKRHVWFGESMTDGFQFEYGGQGSDPADVAIQLTFLRLMSTEASQNITYHCKNSVAYMDQQTGNLKKALLLKGSNEIEIRAEGNSRFTYSVTVDGCTSHTGAWGKTVIEYKTTKSSRLPIIDVAPLDVGAPDQEFGFDVGPVCFL

SEQ ID NO: 59 - protein, 311 aa, synthetic construct
  source 1..311: organism (original language) = 合成构建体
GSNGLPGPIGPPGPRGRTGDAGPVGPPGPPGPPGPPGPPSAGFDFSFLPQPPQEKAHDGGRYYRANDANVVRDRDLEVDTTLKSLSQQIENIRSPEGSRKNPARTCRDLKMCHSDWKSGEYWIDPNQGCNLDAIKVFCNMETGETCVYPTQPSVAQKNWYISKNPKDKRHVWFGESMTDGFQFEYGGQGSDPADVAIQLTFLRLMSTEASQNITYHCKNSVAYMDQQTGNLKKALLLKGSNEIEIRAEGNSRFTYSVTVDGCTSHTGAWGKTVIEYKTTKSSRLPIIDVAPLDVGAPDQEFGFDVGPVCFL

SEQ ID NO: 60 - protein, 234 aa, synthetic construct
  source 1..234: organism (original language) = 合成构建体
DEIMTSLKSVNGQIESLISPDGSRKNPARNCRDLKFCHPELKSGEYWVDPNQGCKLDAIKVFCNMETGETCISANPLNVPRKHWWTDSSAEKKHVWFGESMDGGFQFSYGNPELPEDVLDVQLAFLRLLSSRASQNITYHCKNSIAYMDQASGNVKKALKLMGSNEGEFKAEGNSKFTYTVLEDGCTKHTGEWSKTVFEYRTRKAVRLPIVDIAPYDIGGPDQEFGVDVGPVCF

SEQ ID NO: 61 - protein, 244 aa, synthetic construct
  source 1..244: organism (original language) = 合成构建体
EPMDFKINTDEIMTSLKSVNGQIESLISPDGSRKNPARNCRDLKFCHPELKSGEYWVDPNQGCKLDAIKVFCNMETGETCISANPLNVPRKHWWTDSSAEKKHVWFGESMDGGFQFSYGNPELPEDVLDVQLAFLRLLSSRASQNITYHCKNSIAYMDQASGNVKKALKLMGSNEGEFKAEGNSKFTYTVLEDGCTKHTGEWSKTVFEYRTRKAVRLPIVDIAPYDIGGPDQEFGVDVGPVCFL

SEQ ID NO: 62 - protein, 245 aa, synthetic construct
  source 1..245: organism (original language) = 合成构建体
SEPMDFKINTDEIMTSLKSVNGQIESLISPDGSRKNPARNCRDLKFCHPELKSGEYWVDPNQGCKLDAIKVFCNMETGETCISANPLNVPRKHWWTDSSAEKKHVWFGESMDGGFQFSYGNPELPEDVLDVQLAFLRLLSSRASQNITYHCKNSIAYMDQASGNVKKALKLMGSNEGEFKAEGNSKFTYTVLEDGCTKHTGEWSKTVFEYRTRKAVRLPIVDIAPYDIGGPDQEFGVDVGPVCFL

SEQ ID NO: 63 - protein, 246 aa, synthetic construct
  source 1..246: organism (original language) = 合成构建体
RSEPMDFKINTDEIMTSLKSVNGQIESLISPDGSRKNPARNCRDLKFCHPELKSGEYWVDPNQGCKLDAIKVFCNMETGETCISANPLNVPRKHWWTDSSAEKKHVWFGESMDGGFQFSYGNPELPEDVLDVQLAFLRLLSSRASQNITYHCKNSIAYMDQASGNVKKALKLMGSNEGEFKAEGNSKFTYTVLEDGCTKHTGEWSKTVFEYRTRKAVRLPIVDIAPYDIGGPDQEFGVDVGPVCFL

SEQ ID NO: 64 - protein, 824 aa, synthetic construct
  source 1..824: organism (original language) = 合成构建体
MELLILKANAITTILTAVTFCFASGQNITEEFYQSTCSAVSKGYLSALRTGWYTSVITIELSNIKENKCNGTDAKVKLIKQELDKYKNAVTELQLLMQSTPATNNCACRELPRFMNYTLNNAKKTNVTLSKKCKCCFLGFLLGVGSAIASGVAVSKVLHLEGEVNKIKSALLSTNKAVVSLSNGVSVLTSKVLDLKNYIDKQLLPIVNKQSCSISNIETVIEFQQKNNRLLEITREFSVNAGVTTPVSTYMLTNSELLSLINDMPITNDQKKLMSNNVQIVRQQSYSIMSIIKEEVLAYVVQLPLYGVIDTPCWKLHTSPLCTTNTKEGSNICLTRTDRGWYCDNAGSVSFFPQAETCKVQSNRVFCDTMNSLTLPSEVNLCNVDIFNPKYDCKIMTSKTDVSSSVITSLGAIVSCYGKTKCTASNKNRGIIKTFSNGCDYVSNKGVDTVSVGNTLYYVNKQEGKSLYVKGEPIINFYDPLVFPSDEFDASISQVNEKINQSLAFIRKSDELLRSNGLPGPIGPPGPRGRTGDAGPVGPPGPPGPPGPPGPPSAGFDFSFLPQPPQEKAHDGGRYYRANDANVVRDRDLEVDTTLKSLSQQIENIRSPEGSRKNPARTCRDLKMCHSDWKSGEYWIDPNQGCNLDAIKVFCNMETGETCVYPTQPSVAQKNWYISKNPKDKRHVWFGESMTDGFQFEYGGQGSDPADVAIQLTFLRLMSTEASQNITYHCKNSVAYMDQQTGNLKKALLLQGSNEIEIRAEGNSRFTYSVTVDGCTSHTGAWGKTVIEYKTTKTSRLPIIDVAPLDVGAPDQEFGFDVGPVCFL

SEQ ID NO: 65 - protein, 824 aa, synthetic construct
  source 1..824: organism (original language) = 合成构建体
MELLILKANAITTILTAVTFCFASGQNITEEFYQSTCSAVSKGYLSALRTGWYTSVITIELSNIKENKCNGTDAKVKLIKQELDKYKNAVTELQLLMQSTPATNNRACRELPRFMNYTLNNAKKTNVTLSKKCKCCFLGFLLGVGSAIASGVAVSKVLHLEGEVNKIKSALLSTNKAVVSLSNGVSVLTSKVLDLKNYIDKQLLPIVNKQSCSISNIETVIEFQQKNNRLLEITREFSVNAGVTTPVSTYMLTNSELLSLINDMPITNDQKKLMSNNVQIVRQQSYSIMSIIKEEVLAYVVQLPLYGVIDTPCWKLHTSPLCTTNTKEGSNICLTRTDRGWYCDNAGSVSFFPQAETCKVQSNRVFCDTMNSLTLPSEVNLCNVDIFNPKYDCKIMTSKTDVSSSVITSLGAIVSCYGKTKCTASNKNRGIIKTFSNGCDYVSNKGVDTVSVGNTLYYVNKQEGKSLYVKGEPIINFYDPLVFPSDEFDASISQVNEKINQSLAFIRKSDELLRSNGLPGPIGPPGPRGRTGDAGPVGPPGPPGPPGPPGPPSAGFDFSFLPQPPQEKAHDGGRYYRANDANVVRDRDLEVDTTLKSLSQQIENIRSPEGSRKNPARTCRDLKMCHSDWKSGEYWIDPNQGCNLDAIKVFCNMETGETCVYPTQPSVAQKNWYISKNPKDKRHVWFGESMTDGFQFEYGGQGSDPADVAIQLTFLRLMSTEASQNITYHCKNSVAYMDQQTGNLKKALLLQGSNEIEIRAEGNSRFTYSVTVDGCTSHTGAWGKTVIEYKTTKTSRLPIIDVAPLDVGAPDQEFGFDVGPVCFL

SEQ ID NO: 66 - protein, 824 aa, synthetic construct
  source 1..824: organism (original language) = 合成构建体
MELLILKANAITTILTAVTFCFASGQNITEEFYQSTCSAVSKGYLSALRTGWYTSVITIELSNIKENKCNGTDAKVKLIKQELDKYKNAVTELQLLMQSTPATNNRARRELPRFMNYTLNNAKKTNVTLSKKCKCCFLGFLLGVGSAIASGVAVSKVLHLEGEVNKIKSALLSTNKAVVSLSNGVSVLTSKVLDLKNYIDKQLLPIVNKQSCSISNIETVIEFQQKNNRLLEITREFSVNAGVTTPVSTYMLTNSELLSLINDMPITNDQKKLMSNNVQIVRQQSYSIMSIIKEEVLAYVVQLPLYGVIDTPCWKLHTSPLCTTNTKEGSNICLTRTDRGWYCDNAGSVSFFPQAETCKVQSNRVFCDTMNSLTLPSEVNLCNVDIFNPKYDCKIMTSKTDVSSSVITSLGAIVSCYGKTKCTASNKNRGIIKTFSNGCDYVSNKGVDTVSVGNTLYYVNKQEGKSLYVKGEPIINFYDPLVFPSDEFDASISQVNEKINQSLAFIRKSDELLRSNGLPGPIGPPGPRGRTGDAGPVGPPGPPGPPGPPGPPSAGFDFSFLPQPPQEKAHDGGRYYRANDANVVRDRDLEVDTTLKSLSQQIENIRSPEGSRKNPARTCRDLKMCHSDWKSGEYWIDPNQGCNLDAIKVFCNMETGETCVYPTQPSVAQKNWYISKNPKDKRHVWFGESMTDGFQFEYGGQGSDPADVAIQLTFLRLMSTEASQNITYHCKNSVAYMDQQTGNLKKALLLQGSNEIEIRAEGNSRFTYSVTVDGCTSHTGAWGKTVIEYKTTKTSRLPIIDVAPLDVGAPDQEFGFDVGPVCFL

SEQ ID NO: 67 - protein, 824 aa, synthetic construct
  source 1..824: organism (original language) = 合成构建体
MELLILKANAITTILTAVTFCFASGQNITEEFYQSTCSAVSKGYLSALRTGWYTSVITIELSNIKENKCNGTDAKVKLIKQELDKYKNAVTELQLLMQSTPATNNRARRELPRFMNYTLNNAKKTNVTLSKKRKCCFLGFLLGVGSAIASGVAVSKVLHLEGEVNKIKSALLSTNKAVVSLSNGVSVLTSKVLDLKNYIDKQLLPIVNKQSCSISNIETVIEFQQKNNRLLEITREFSVNAGVTTPVSTYMLTNSELLSLINDMPITNDQKKLMSNNVQIVRQQSYSIMSIIKEEVLAYVVQLPLYGVIDTPCWKLHTSPLCTTNTKEGSNICLTRTDRGWYCDNAGSVSFFPQAETCKVQSNRVFCDTMNSLTLPSEVNLCNVDIFNPKYDCKIMTSKTDVSSSVITSLGAIVSCYGKTKCTASNKNRGIIKTFSNGCDYVSNKGVDTVSVGNTLYYVNKQEGKSLYVKGEPIINFYDPLVFPSDEFDASISQVNEKINQSLAFIRKSDELLRSNGLPGPIGPPGPRGRTGDAGPVGPPGPPGPPGPPGPPSAGFDFSFLPQPPQEKAHDGGRYYRANDANVVRDRDLEVDTTLKSLSQQIENIRSPEGSRKNPARTCRDLKMCHSDWKSGEYWIDPNQGCNLDAIKVFCNMETGETCVYPTQPSVAQKNWYISKNPKDKRHVWFGESMTDGFQFEYGGQGSDPADVAIQLTFLRLMSTEASQNITYHCKNSVAYMDQQTGNLKKALLLQGSNEIEIRAEGNSRFTYSVTVDGCTSHTGAWGKTVIEYKTTKTSRLPIIDVAPLDVGAPDQEFGFDVGPVCFL

SEQ ID NO: 68 - protein, 799 aa, synthetic construct
  source 1..799: organism (original language) = 合成构建体
QNITEEFYQSTCSAVSKGYLSALRTGWYTSVITIELSNIKENKCNGTDAKVKLIKQELDKYKNAVTELQLLMQSTPATNNCACRELPRFMNYTLNNAKKTNVTLSKKCKCCFLGFLLGVGSAIASGVAVSKVLHLEGEVNKIKSALLSTNKAVVSLSNGVSVLTSKVLDLKNYIDKQLLPIVNKQSCSISNIETVIEFQQKNNRLLEITREFSVNAGVTTPVSTYMLTNSELLSLINDMPITNDQKKLMSNNVQIVRQQSYSIMSIIKEEVLAYVVQLPLYGVIDTPCWKLHTSPLCTTNTKEGSNICLTRTDRGWYCDNAGSVSFFPQAETCKVQSNRVFCDTMNSLTLPSEVNLCNVDIFNPKYDCKIMTSKTDVSSSVITSLGAIVSCYGKTKCTASNKNRGIIKTFSNGCDYVSNKGVDTVSVGNTLYYVNKQEGKSLYVKGEPIINFYDPLVFPSDEFDASISQVNEKINQSLAFIRKSDELLRSNGLPGPIGPPGPRGRTGDAGPVGPPGPPGPPGPPGPPSAGFDFSFLPQPPQEKAHDGGRYYRANDANVVRDRDLEVDTTLKSLSQQIENIRSPEGSRKNPARTCRDLKMCHSDWKSGEYWIDPNQGCNLDAIKVFCNMETGETCVYPTQPSVAQKNWYISKNPKDKRHVWFGESMTDGFQFEYGGQGSDPADVAIQLTFLRLMSTEASQNITYHCKNSVAYMDQQTGNLKKALLLQGSNEIEIRAEGNSRFTYSVTVDGCTSHTGAWGKTVIEYKTTKTSRLPIIDVAPLDVGAPDQEFGFDVGPVCFL

SEQ ID NO: 69 - protein, 799 aa, synthetic construct
  source 1..799: organism (original language) = 合成构建体
QNITEEFYQSTCSAVSKGYLSALRTGWYTSVITIELSNIKENKCNGTDAKVKLIKQELDKYKNAVTELQLLMQSTPATNNRACRELPRFMNYTLNNAKKTNVTLSKKCKCCFLGFLLGVGSAIASGVAVSKVLHLEGEVNKIKSALLSTNKAVVSLSNGVSVLTSKVLDLKNYIDKQLLPIVNKQSCSISNIETVIEFQQKNNRLLEITREFSVNAGVTTPVSTYMLTNSELLSLINDMPITNDQKKLMSNNVQIVRQQSYSIMSIIKEEVLAYVVQLPLYGVIDTPCWKLHTSPLCTTNTKEGSNICLTRTDRGWYCDNAGSVSFFPQAETCKVQSNRVFCDTMNSLTLPSEVNLCNVDIFNPKYDCKIMTSKTDVSSSVITSLGAIVSCYGKTKCTASNKNRGIIKTFSNGCDYVSNKGVDTVSVGNTLYYVNKQEGKSLYVKGEPIINFYDPLVFPSDEFDASISQVNEKINQSLAFIRKSDELLRSNGLPGPIGPPGPRGRTGDAGPVGPPGPPGPPGPPGPPSAGFDFSFLPQPPQEKAHDGGRYYRANDANVVRDRDLEVDTTLKSLSQQIENIRSPEGSRKNPARTCRDLKMCHSDWKSGEYWIDPNQGCNLDAIKVFCNMETGETCVYPTQPSVAQKNWYISKNPKDKRHVWFGESMTDGFQFEYGGQGSDPADVAIQLTFLRLMSTEASQNITYHCKNSVAYMDQQTGNLKKALLLQGSNEIEIRAEGNSRFTYSVTVDGCTSHTGAWGKTVIEYKTTKTSRLPIIDVAPLDVGAPDQEFGFDVGPVCFL

SEQ ID NO: 70 - protein, 799 aa, synthetic construct
  source 1..799: organism (original language) = 合成构建体
QNITEEFYQSTCSAVSKGYLSALRTGWYTSVITIELSNIKENKCNGTDAKVKLIKQELDKYKNAVTELQLLMQSTPATNNRARRELPRFMNYTLNNAKKTNVTLSKKCKCCFLGFLLGVGSAIASGVAVSKVLHLEGEVNKIKSALLSTNKAVVSLSNGVSVLTSKVLDLKNYIDKQLLPIVNKQSCSISNIETVIEFQQKNNRLLEITREFSVNAGVTTPVSTYMLTNSELLSLINDMPITNDQKKLMSNNVQIVRQQSYSIMSIIKEEVLAYVVQLPLYGVIDTPCWKLHTSPLCTTNTKEGSNICLTRTDRGWYCDNAGSVSFFPQAETCKVQSNRVFCDTMNSLTLPSEVNLCNVDIFNPKYDCKIMTSKTDVSSSVITSLGAIVSCYGKTKCTASNKNRGIIKTFSNGCDYVSNKGVDTVSVGNTLYYVNKQEGKSLYVKGEPIINFYDPLVFPSDEFDASISQVNEKINQSLAFIRKSDELLRSNGLPGPIGPPGPRGRTGDAGPVGPPGPPGPPGPPGPPSAGFDFSFLPQPPQEKAHDGGRYYRANDANVVRDRDLEVDTTLKSLSQQIENIRSPEGSRKNPARTCRDLKMCHSDWKSGEYWIDPNQGCNLDAIKVFCNMETGETCVYPTQPSVAQKNWYISKNPKDKRHVWFGESMTDGFQFEYGGQGSDPADVAIQLTFLRLMSTEASQNITYHCKNSVAYMDQQTGNLKKALLLQGSNEIEIRAEGNSRFTYSVTVDGCTSHTGAWGKTVIEYKTTKTSRLPIIDVAPLDVGAPDQEFGFDVGPVCFL

SEQ ID NO: 71 - protein, 799 aa, synthetic construct
  source 1..799: organism (original language) = 合成构建体
QNITEEFYQSTCSAVSKGYLSALRTGWYTSVITIELSNIKENKCNGTDAKVKLIKQELDKYKNAVTELQLLMQSTPATNNRARRELPRFMNYTLNNAKKTNVTLSKKRKCCFLGFLLGVGSAIASGVAVSKVLHLEGEVNKIKSALLSTNKAVVSLSNGVSVLTSKVLDLKNYIDKQLLPIVNKQSCSISNIETVIEFQQKNNRLLEITREFSVNAGVTTPVSTYMLTNSELLSLINDMPITNDQKKLMSNNVQIVRQQSYSIMSIIKEEVLAYVVQLPLYGVIDTPCWKLHTSPLCTTNTKEGSNICLTRTDRGWYCDNAGSVSFFPQAETCKVQSNRVFCDTMNSLTLPSEVNLCNVDIFNPKYDCKIMTSKTDVSSSVITSLGAIVSCYGKTKCTASNKNRGIIKTFSNGCDYVSNKGVDTVSVGNTLYYVNKQEGKSLYVKGEPIINFYDPLVFPSDEFDASISQVNEKINQSLAFIRKSDELLRSNGLPGPIGPPGPRGRTGDAGPVGPPGPPGPPGPPGPPSAGFDFSFLPQPPQEKAHDGGRYYRANDANVVRDRDLEVDTTLKSLSQQIENIRSPEGSRKNPARTCRDLKMCHSDWKSGEYWIDPNQGCNLDAIKVFCNMETGETCVYPTQPSVAQKNWYISKNPKDKRHVWFGESMTDGFQFEYGGQGSDPADVAIQLTFLRLMSTEASQNITYHCKNSVAYMDQQTGNLKKALLLQGSNEIEIRAEGNSRFTYSVTVDGCTSHTGAWGKTVIEYKTTKTSRLPIIDVAPLDVGAPDQEFGFDVGPVCFL

SEQ ID NO: 72 - protein, 513 aa, synthetic construct
  source 1..513: organism (original language) = 合成构建体
MELLILKANAITTILTAVTFCFASGQNITEEFYQSTCSAVSKGYLSALRTGWYTSVITIELSNIKENKCNGTDAKVKLIKQELDKYKNAVTELQLLMQSTPATNNCACRELPRFMNYTLNNAKKTNVTLSKKCKCCFLGFLLGVGSAIASGVAVSKVLHLEGEVNKIKSALLSTNKAVVSLSNGVSVLTSKVLDLKNYIDKQLLPIVNKQSCSISNIETVIEFQQKNNRLLEITREFSVNAGVTTPVSTYMLTNSELLSLINDMPITNDQKKLMSNNVQIVRQQSYSIMSIIKEEVLAYVVQLPLYGVIDTPCWKLHTSPLCTTNTKEGSNICLTRTDRGWYCDNAGSVSFFPQAETCKVQSNRVFCDTMNSLTLPSEVNLCNVDIFNPKYDCKIMTSKTDVSSSVITSLGAIVSCYGKTKCTASNKNRGIIKTFSNGCDYVSNKGVDTVSVGNTLYYVNKQEGKSLYVKGEPIINFYDPLVFPSDEFDASISQVNEKINQSLAFIRKSDELL

SEQ ID NO: 73 - protein, 513 aa, synthetic construct
  source 1..513: organism (original language) = 合成构建体
MELLILKANAITTILTAVTFCFASGQNITEEFYQSTCSAVSKGYLSALRTGWYTSVITIELSNIKENKCNGTDAKVKLIKQELDKYKNAVTELQLLMQSTPATNNRACRELPRFMNYTLNNAKKTNVTLSKKCKCCFLGFLLGVGSAIASGVAVSKVLHLEGEVNKIKSALLSTNKAVVSLSNGVSVLTSKVLDLKNYIDKQLLPIVNKQSCSISNIETVIEFQQKNNRLLEITREFSVNAGVTTPVSTYMLTNSELLSLINDMPITNDQKKLMSNNVQIVRQQSYSIMSIIKEEVLAYVVQLPLYGVIDTPCWKLHTSPLCTTNTKEGSNICLTRTDRGWYCDNAGSVSFFPQAETCKVQSNRVFCDTMNSLTLPSEVNLCNVDIFNPKYDCKIMTSKTDVSSSVITSLGAIVSCYGKTKCTASNKNRGIIKTFSNGCDYVSNKGVDTVSVGNTLYYVNKQEGKSLYVKGEPIINFYDPLVFPSDEFDASISQVNEKINQSLAFIRKSDELL

SEQ ID NO: 74 - protein, 513 aa, synthetic construct
  source 1..513: organism (original language) = 合成构建体
MELLILKANAITTILTAVTFCFASGQNITEEFYQSTCSAVSKGYLSALRTGWYTSVITIELSNIKENKCNGTDAKVKLIKQELDKYKNAVTELQLLMQSTPATNNRARRELPRFMNYTLNNAKKTNVTLSKKCKCCFLGFLLGVGSAIASGVAVSKVLHLEGEVNKIKSALLSTNKAVVSLSNGVSVLTSKVLDLKNYIDKQLLPIVNKQSCSISNIETVIEFQQKNNRLLEITREFSVNAGVTTPVSTYMLTNSELLSLINDMPITNDQKKLMSNNVQIVRQQSYSIMSIIKEEVLAYVVQLPLYGVIDTPCWKLHTSPLCTTNTKEGSNICLTRTDRGWYCDNAGSVSFFPQAETCKVQSNRVFCDTMNSLTLPSEVNLCNVDIFNPKYDCKIMTSKTDVSSSVITSLGAIVSCYGKTKCTASNKNRGIIKTFSNGCDYVSNKGVDTVSVGNTLYYVNKQEGKSLYVKGEPIINFYDPLVFPSDEFDASISQVNEKINQSLAFIRKSDELL

SEQ ID NO: 75 - protein, 513 aa, synthetic construct
  source 1..513: organism (original language) = 合成构建体
MELLILKANAITTILTAVTFCFASGQNITEEFYQSTCSAVSKGYLSALRTGWYTSVITIELSNIKENKCNGTDAKVKLIKQELDKYKNAVTELQLLMQSTPATNNRARRELPRFMNYTLNNAKKTNVTLSKKRKCCFLGFLLGVGSAIASGVAVSKVLHLEGEVNKIKSALLSTNKAVVSLSNGVSVLTSKVLDLKNYIDKQLLPIVNKQSCSISNIETVIEFQQKNNRLLEITREFSVNAGVTTPVSTYMLTNSELLSLINDMPITNDQKKLMSNNVQIVRQQSYSIMSIIKEEVLAYVVQLPLYGVIDTPCWKLHTSPLCTTNTKEGSNICLTRTDRGWYCDNAGSVSFFPQAETCKVQSNRVFCDTMNSLTLPSEVNLCNVDIFNPKYDCKIMTSKTDVSSSVITSLGAIVSCYGKTKCTASNKNRGIIKTFSNGCDYVSNKGVDTVSVGNTLYYVNKQEGKSLYVKGEPIINFYDPLVFPSDEFDASISQVNEKINQSLAFIRKSDELL

SEQ ID NO: 76 - protein, 488 aa, synthetic construct
  source 1..488: organism (original language) = 合成构建体
QNITEEFYQSTCSAVSKGYLSALRTGWYTSVITIELSNIKENKCNGTDAKVKLIKQELDKYKNAVTELQLLMQSTPATNNCACRELPRFMNYTLNNAKKTNVTLSKKCKCCFLGFLLGVGSAIASGVAVSKVLHLEGEVNKIKSALLSTNKAVVSLSNGVSVLTSKVLDLKNYIDKQLLPIVNKQSCSISNIETVIEFQQKNNRLLEITREFSVNAGVTTPVSTYMLTNSELLSLINDMPITNDQKKLMSNNVQIVRQQSYSIMSIIKEEVLAYVVQLPLYGVIDTPCWKLHTSPLCTTNTKEGSNICLTRTDRGWYCDNAGSVSFFPQAETCKVQSNRVFCDTMNSLTLPSEVNLCNVDIFNPKYDCKIMTSKTDVSSSVITSLGAIVSCYGKTKCTASNKNRGIIKTFSNGCDYVSNKGVDTVSVGNTLYYVNKQEGKSLYVKGEPIINFYDPLVFPSDEFDASISQVNEKINQSLAFIRKSDELL

SEQ ID NO: 77 - protein, 488 aa, synthetic construct
  source 1..488: organism (original language) = 合成构建体
QNITEEFYQSTCSAVSKGYLSALRTGWYTSVITIELSNIKENKCNGTDAKVKLIKQELDKYKNAVTELQLLMQSTPATNNRACRELPRFMNYTLNNAKKTNVTLSKKCKCCFLGFLLGVGSAIASGVAVSKVLHLEGEVNKIKSALLSTNKAVVSLSNGVSVLTSKVLDLKNYIDKQLLPIVNKQSCSISNIETVIEFQQKNNRLLEITREFSVNAGVTTPVSTYMLTNSELLSLINDMPITNDQKKLMSNNVQIVRQQSYSIMSIIKEEVLAYVVQLPLYGVIDTPCWKLHTSPLCTTNTKEGSNICLTRTDRGWYCDNAGSVSFFPQAETCKVQSNRVFCDTMNSLTLPSEVNLCNVDIFNPKYDCKIMTSKTDVSSSVITSLGAIVSCYGKTKCTASNKNRGIIKTFSNGCDYVSNKGVDTVSVGNTLYYVNKQEGKSLYVKGEPIINFYDPLVFPSDEFDASISQVNEKINQSLAFIRKSDELL

SEQ ID NO: 78 - protein, 488 aa, synthetic construct
  source 1..488: organism (original language) = 合成构建体
QNITEEFYQSTCSAVSKGYLSALRTGWYTSVITIELSNIKENKCNGTDAKVKLIKQELDKYKNAVTELQLLMQSTPATNNRARRELPRFMNYTLNNAKKTNVTLSKKCKCCFLGFLLGVGSAIASGVAVSKVLHLEGEVNKIKSALLSTNKAVVSLSNGVSVLTSKVLDLKNYIDKQLLPIVNKQSCSISNIETVIEFQQKNNRLLEITREFSVNAGVTTPVSTYMLTNSELLSLINDMPITNDQKKLMSNNVQIVRQQSYSIMSIIKEEVLAYVVQLPLYGVIDTPCWKLHTSPLCTTNTKEGSNICLTRTDRGWYCDNAGSVSFFPQAETCKVQSNRVFCDTMNSLTLPSEVNLCNVDIFNPKYDCKIMTSKTDVSSSVITSLGAIVSCYGKTKCTASNKNRGIIKTFSNGCDYVSNKGVDTVSVGNTLYYVNKQEGKSLYVKGEPIINFYDPLVFPSDEFDASISQVNEKINQSLAFIRKSDELL

SEQ ID NO: 79 - protein, 488 aa, synthetic construct
  source 1..488: organism (original language) = 合成构建体
QNITEEFYQSTCSAVSKGYLSALRTGWYTSVITIELSNIKENKCNGTDAKVKLIKQELDKYKNAVTELQLLMQSTPATNNRARRELPRFMNYTLNNAKKTNVTLSKKRKCCFLGFLLGVGSAIASGVAVSKVLHLEGEVNKIKSALLSTNKAVVSLSNGVSVLTSKVLDLKNYIDKQLLPIVNKQSCSISNIETVIEFQQKNNRLLEITREFSVNAGVTTPVSTYMLTNSELLSLINDMPITNDQKKLMSNNVQIVRQQSYSIMSIIKEEVLAYVVQLPLYGVIDTPCWKLHTSPLCTTNTKEGSNICLTRTDRGWYCDNAGSVSFFPQAETCKVQSNRVFCDTMNSLTLPSEVNLCNVDIFNPKYDCKIMTSKTDVSSSVITSLGAIVSCYGKTKCTASNKNRGIIKTFSNGCDYVSNKGVDTVSVGNTLYYVNKQEGKSLYVKGEPIINFYDPLVFPSDEFDASISQVNEKINQSLAFIRKSDELL

SEQ ID NO: 80 - protein, 824 aa, synthetic construct
  source 1..824: organism (original language) = 合成构建体
MELLILKANAITTILTAVTFCFASGQNITEEFYQSTCSAVSKGYLSALRTGWYTSVITIELSNIKENKCNGTDAKVKLIKQELDKYKNAVTELQLLMQSTPATNNAAARELPRFMNYTLNNAKKTNVTLSKKAKAAFLGFLLGVGSAIASGVAVSKVLHLEGEVNKIKSALLSTNKAVVSLSNGVSVLTSKVLDLKNYIDKQLLPIVNKQSCSISNIETVIEFQQKNNRLLEITREFSVNAGVTTPVSTYMLTNSELLSLINDMPITNDQKKLMSNNVQIVRQQSYSIMSIIKEEVLAYVVQLPLYGVIDTPCWKLHTSPLCTTNTKEGSNICLTRTDRGWYCDNAGSVSFFPQAETCKVQSNRVFCDTMNSLTLPSEVNLCNVDIFNPKYDCKIMTSKTDVSSSVITSLGAIVSCYGKTKCTASNKNRGIIKTFSNGCDYVSNKGVDTVSVGNTLYYVNKQEGKSLYVKGEPIINFYDPLVFPSDEFDASISQVNEKINQSLAFIRKSDELLRSNGLPGPIGPPGPRGRTGDAGPVGPPGPPGPPGPPGPPSAGFDFSFLPQPPQEKAHDGGRYYRANDANVVRDRDLEVDTTLKSLSQQIENIRSPEGSRKNPARTCRDLKMCHSDWKSGEYWIDPNQGCNLDAIKVFCNMETGETCVYPTQPSVAQKNWYISKNPKDKRHVWFGESMTDGFQFEYGGQGSDPADVAIQLTFLRLMSTEASQNITYHCKNSVAYMDQQTGNLKKALLLQGSNEIEIRAEGNSRFTYSVTVDGCTSHTGAWGKTVIEYKTTKTSRLPIIDVAPLDVGAPDQEFGFDVGPVCFL

SEQ ID NO: 81 - protein, 824 aa, synthetic construct
  source 1..824: organism (original language) = 合成构建体
MELLILKANAITTILTAVTFCFASGQNITEEFYQSTCSAVSKGYLSALRTGWYTSVITIELSNIKENKCNGTDAKVKLIKQELDKYKNAVTELQLLMQSTPATNNTATRELPRFMNYTLNNAKKTNVTLSKKTKTTFLGFLLGVGSAIASGVAVSKVLHLEGEVNKIKSALLSTNKAVVSLSNGVSVLTSKVLDLKNYIDKQLLPIVNKQSCSISNIETVIEFQQKNNRLLEITREFSVNAGVTTPVSTYMLTNSELLSLINDMPITNDQKKLMSNNVQIVRQQSYSIMSIIKEEVLAYVVQLPLYGVIDTPCWKLHTSPLCTTNTKEGSNICLTRTDRGWYCDNAGSVSFFPQAETCKVQSNRVFCDTMNSLTLPSEVNLCNVDIFNPKYDCKIMTSKTDVSSSVITSLGAIVSCYGKTKCTASNKNRGIIKTFSNGCDYVSNKGVDTVSVGNTLYYVNKQEGKSLYVKGEPIINFYDPLVFPSDEFDASISQVNEKINQSLAFIRKSDELLRSNGLPGPIGPPGPRGRTGDAGPVGPPGPPGPPGPPGPPSAGFDFSFLPQPPQEKAHDGGRYYRANDANVVRDRDLEVDTTLKSLSQQIENIRSPEGSRKNPARTCRDLKMCHSDWKSGEYWIDPNQGCNLDAIKVFCNMETGETCVYPTQPSVAQKNWYISKNPKDKRHVWFGESMTDGFQFEYGGQGSDPADVAIQLTFLRLMSTEASQNITYHCKNSVAYMDQQTGNLKKALLLQGSNEIEIRAEGNSRFTYSVTVDGCTSHTGAWGKTVIEYKTTKTSRLPIIDVAPLDVGAPDQEFGFDVGPVCFL

SEQ ID NO: 82 - protein, 824 aa, synthetic construct
  source 1..824: organism (original language) = 合成构建体
MELLILKANAITTILTAVTFCFASGQNITEEFYQSTCSAVSKGYLSALRTGWYTSVITIELSNIKENKCNGTDAKVKLIKQELDKYKNAVTELQLLMQSTPATNNYAYRELPRFMNYTLNNAKKTNVTLSKKYKYYFLGFLLGVGSAIASGVAVSKVLHLEGEVNKIKSALLSTNKAVVSLSNGVSVLTSKVLDLKNYIDKQLLPIVNKQSCSISNIETVIEFQQKNNRLLEITREFSVNAGVTTPVSTYMLTNSELLSLINDMPITNDQKKLMSNNVQIVRQQSYSIMSIIKEEVLAYVVQLPLYGVIDTPCWKLHTSPLCTTNTKEGSNICLTRTDRGWYCDNAGSVSFFPQAETCKVQSNRVFCDTMNSLTLPSEVNLCNVDIFNPKYDCKIMTSKTDVSSSVITSLGAIVSCYGKTKCTASNKNRGIIKTFSNGCDYVSNKGVDTVSVGNTLYYVNKQEGKSLYVKGEPIINFYDPLVFPSDEFDASISQVNEKINQSLAFIRKSDELLRSNGLPGPIGPPGPRGRTGDAGPVGPPGPPGPPGPPGPPSAGFDFSFLPQPPQEKAHDGGRYYRANDANVVRDRDLEVDTTLKSLSQQIENIRSPEGSRKNPARTCRDLKMCHSDWKSGEYWIDPNQGCNLDAIKVFCNMETGETCVYPTQPSVAQKNWYISKNPKDKRHVWFGESMTDGFQFEYGGQGSDPADVAIQLTFLRLMSTEASQNITYHCKNSVAYMDQQTGNLKKALLLQGSNEIEIRAEGNSRFTYSVTVDGCTSHTGAWGKTVIEYKTTKTSRLPIIDVAPLDVGAPDQEFGFDVGPVCFL

SEQ ID NO: 83 - protein, 824 aa, synthetic construct
  source 1..824: organism (original language) = 合成构建体
MELLILKANAITTILTAVTFCFASGQNITEEFYQSTCSAVSKGYLSALRTGWYTSVITIELSNIKENKCNGTDAKVKLIKQELDKYKNAVTELQLLMQSTPATNNGAGRELPRFMNYTLNNAKKTNVTLSKKGKGGFLGFLLGVGSAIASGVAVSKVLHLEGEVNKIKSALLSTNKAVVSLSNGVSVLTSKVLDLKNYIDKQLLPIVNKQSCSISNIETVIEFQQKNNRLLEITREFSVNAGVTTPVSTYMLTNSELLSLINDMPITNDQKKLMSNNVQIVRQQSYSIMSIIKEEVLAYVVQLPLYGVIDTPCWKLHTSPLCTTNTKEGSNICLTRTDRGWYCDNAGSVSFFPQAETCKVQSNRVFCDTMNSLTLPSEVNLCNVDIFNPKYDCKIMTSKTDVSSSVITSLGAIVSCYGKTKCTASNKNRGIIKTFSNGCDYVSNKGVDTVSVGNTLYYVNKQEGKSLYVKGEPIINFYDPLVFPSDEFDASISQVNEKINQSLAFIRKSDELLRSNGLPGPIGPPGPRGRTGDAGPVGPPGPPGPPGPPGPPSAGFDFSFLPQPPQEKAHDGGRYYRANDANVVRDRDLEVDTTLKSLSQQIENIRSPEGSRKNPARTCRDLKMCHSDWKSGEYWIDPNQGCNLDAIKVFCNMETGETCVYPTQPSVAQKNWYISKNPKDKRHVWFGESMTDGFQFEYGGQGSDPADVAIQLTFLRLMSTEASQNITYHCKNSVAYMDQQTGNLKKALLLQGSNEIEIRAEGNSRFTYSVTVDGCTSHTGAWGKTVIEYKTTKTSRLPIIDVAPLDVGAPDQEFGFDVGPVCFL

SEQ ID NO: 84 - protein, 824 aa, synthetic construct
  source 1..824: organism (original language) = 合成构建体
MELLILKANAITTILTAVTFCFASGQNITEEFYQSTCSAVSKGYLSALRTGWYTSVITIELSNIKENKCNGTDAKVKLIKQELDKYKNAVTELQLLMQSTPATNNSASRELPRFMNYTLNNAKKTNVTLSKKSKSSFLGFLLGVGSAIASGVAVSKVLHLEGEVNKIKSALLSTNKAVVSLSNGVSVLTSKVLDLKNYIDKQLLPIVNKQSCSISNIETVIEFQQKNNRLLEITREFSVNAGVTTPVSTYMLTNSELLSLINDMPITNDQKKLMSNNVQIVRQQSYSIMSIIKEEVLAYVVQLPLYGVIDTPCWKLHTSPLCTTNTKEGSNICLTRTDRGWYCDNAGSVSFFPQAETCKVQSNRVFCDTMNSLTLPSEVNLCNVDIFNPKYDCKIMTSKTDVSSSVITSLGAIVSCYGKTKCTASNKNRGIIKTFSNGCDYVSNKGVDTVSVGNTLYYVNKQEGKSLYVKGEPIINFYDPLVFPSDEFDASISQVNEKINQSLAFIRKSDELLRSNGLPGPIGPPGPRGRTGDAGPVGPPGPPGPPGPPGPPSAGFDFSFLPQPPQEKAHDGGRYYRANDANVVRDRDLEVDTTLKSLSQQIENIRSPEGSRKNPARTCRDLKMCHSDWKSGEYWIDPNQGCNLDAIKVFCNMETGETCVYPTQPSVAQKNWYISKNPKDKRHVWFGESMTDGFQFEYGGQGSDPADVAIQLTFLRLMSTEASQNITYHCKNSVAYMDQQTGNLKKALLLQGSNEIEIRAEGNSRFTYSVTVDGCTSHTGAWGKTVIEYKTTKTSRLPIIDVAPLDVGAPDQEFGFDVGPVCFL